European Patent Specification EP 3 774 917 B1, published October 29, 2025. Title: Single-domain antibodies against LAG-3 and uses thereof. Applicant: Nanjing Legend Biotech Co., Ltd. Application Not Yet Assigned. The sequence listing filed with the application follows.

SEQUENCE LISTING (446 sequences)

SEQ ID NO: 1 - protein, 25 aa, Artificial Sequence
  Synthetic Construct
QVQLAESGGGSVHAGGSLRLSCVVS

SEQ ID NO: 2 - protein, 25 aa, Artificial Sequence
  Synthetic Construct
EVQLVESGGGSVQAGGSLRLSCAAS

SEQ ID NO: 3 - protein, 25 aa, Artificial Sequence
  Synthetic Construct
QVQLAESGGGSVQAGGSLRLSCAAS

SEQ ID NO: 4 - protein, 25 aa, Artificial Sequence
  Synthetic Construct
EVQLAESGGGSVQAGGSLRLSCAAS

SEQ ID NO: 5 - protein, 25 aa, Artificial Sequence
  Synthetic Construct
QVHLMESGGGSVQVGGSLRLSCAAS

SEQ ID NO: 6 - protein, 25 aa, Artificial Sequence
  Synthetic Construct
EVQLVESGGGLVQAGGSLRLSCTAS

SEQ ID NO: 7 - protein, 25 aa, Artificial Sequence
  Synthetic Construct
QVQLVESGGGSVQAGGSLRLSCAAS

SEQ ID NO: 8 - protein, 25 aa, Artificial Sequence
  Synthetic Construct
EVQLVESGGGSVQAGGSLRLSCAAS

SEQ ID NO: 9 - protein, 25 aa, Artificial Sequence [sequence omitted]

SEQ ID NO: 10 - protein, 25 aa, Artificial Sequence [sequence omitted]

SEQ ID NO: 11 - protein, 25 aa, Artificial Sequence [sequence omitted]

SEQ ID NO: 12 - protein, 25 aa, Artificial Sequence [sequence omitted]

SEQ ID NO: 13 - protein, 25 aa, Artificial Sequence [sequence omitted]

SEQ ID NO: 14 - protein, 25 aa, Artificial Sequence [sequence omitted]

SEQ ID NO: 15 - protein, 25 aa, Artificial Sequence [sequence omitted]

SEQ ID NO: 16 - protein, 25 aa, Artificial Sequence [sequence omitted]

SEQ ID NO: 17 - protein, 25 aa, Artificial Sequence [sequence omitted]

SEQ ID NO: 18 - protein, 25 aa, Artificial Sequence [sequence omitted]

SEQ ID NO: 19 - protein, 25 aa, Artificial Sequence [sequence omitted]

SEQ ID NO: 20 - protein, 25 aa, Artificial Sequence [sequence omitted]

SEQ ID NO: 21 - protein, 25 aa, Artificial Sequence [sequence omitted]

SEQ ID NO: 22 - protein, 25 aa, Artificial Sequence [sequence omitted]

SEQ ID NO: 23 - protein, 25 aa, Artificial Sequence [sequence omitted]

SEQ ID NO: 24 - protein, 25 aa, Artificial Sequence [sequence omitted]

SEQ ID NO: 25 - protein, 25 aa, Artificial Sequence [sequence omitted]

SEQ ID NO: 26 - protein, 25 aa, Artificial Sequence [sequence omitted]

SEQ ID NO: 27 - protein, 25 aa, Artificial Sequence [sequence omitted]

SEQ ID NO: 28 - protein, 25 aa, Artificial Sequence [sequence omitted]

SEQ ID NO: 29 - protein, 25 aa, Artificial Sequence [sequence omitted]

SEQ ID NO: 30 - protein, 25 aa, Artificial Sequence [sequence omitted]

SEQ ID NO: 31 - protein, 25 aa, Artificial Sequence [sequence omitted]

SEQ ID NO: 32 - protein, 25 aa, Artificial Sequence [sequence omitted]

SEQ ID NO: 33 - protein, 25 aa, Artificial Sequence [sequence omitted]

SEQ ID NO: 34 - protein, 25 aa, Artificial Sequence [sequence omitted]

SEQ ID NO: 35 - protein, 25 aa, Artificial Sequence [sequence omitted]

SEQ ID NO: 36 - protein, 25 aa, Artificial Sequence [sequence omitted]

SEQ ID NO: 37 - protein, 25 aa, Artificial Sequence [sequence omitted]

SEQ ID NO: 38 - protein, 25 aa, Artificial Sequence [sequence omitted]

SEQ ID NO: 39 - protein, 10 aa, Artificial Sequence
  Synthetic Construct
EYTFSSDSMG

SEQ ID NO: 40 - protein, 10 aa, Artificial Sequence
  Synthetic Construct
GYIISSYCMG

SEQ ID NO: 41 - protein, 10 aa, Artificial Sequence
  Synthetic Construct
GYTISSYCMG

SEQ ID NO: 42 - protein, 10 aa, Artificial Sequence
  Synthetic Construct
GYTYGGYCMG

SEQ ID NO: 43 - protein, 10 aa, Artificial Sequence
  Synthetic Construct
GYTVSSYCMG

SEQ ID NO: 44 - protein, 10 aa, Artificial Sequence
  Synthetic Construct
GLTFDDYAMG

SEQ ID NO: 45 - protein, 10 aa, Artificial Sequence
  Synthetic Construct
GYTLSSYCMG

SEQ ID NO: 46 - protein, 10 aa, Artificial Sequence
  Synthetic Construct
GYIISSYCMG

SEQ ID NO: 47 - protein, 10 aa, Artificial Sequence
  Synthetic Construct
GYIISSYCMG

SEQ ID NO: 48 - protein, 10 aa, Artificial Sequence
  Synthetic Construct
GYIISSYCMG

SEQ ID NO: 49 - protein, 10 aa, Artificial Sequence
  Synthetic Construct
GYIISSYCMG

SEQ ID NO: 50 - protein, 10 aa, Artificial Sequence
  Synthetic Construct
GYIISSYCMG

SEQ ID NO: 51 - protein, 10 aa, Artificial Sequence
  Synthetic Construct
GYIISSYCMG

SEQ ID NO: 52 - protein, 10 aa, Artificial Sequence
  Synthetic Construct
GYIISSYCMG

SEQ ID NO: 53 - protein, 10 aa, Artificial Sequence
  Synthetic Construct
GYIISSYCMG

SEQ ID NO: 54 - protein, 10 aa, Artificial Sequence
  Synthetic Construct
GYIISSYCMG

SEQ ID NO: 55 - protein, 10 aa, Artificial Sequence
  Synthetic Construct
GYTISSYCMG

SEQ ID NO: 56 - protein, 10 aa, Artificial Sequence
  Synthetic Construct
GYTISSYCMG

SEQ ID NO: 57 - protein, 10 aa, Artificial Sequence
  Synthetic Construct
GYTISSYCMG

SEQ ID NO: 58 - protein, 10 aa, Artificial Sequence
  Synthetic Construct
GYTISSYCMG

SEQ ID NO: 59 - protein, 10 aa, Artificial Sequence
  Synthetic Construct
GYTISSYCMG

SEQ ID NO: 60 - protein, 10 aa, Artificial Sequence
  Synthetic Construct
GYTISSYCMG

SEQ ID NO: 61 - protein, 10 aa, Artificial Sequence
  Synthetic Construct
GYTISSYCMG

SEQ ID NO: 62 - protein, 10 aa, Artificial Sequence
  Synthetic Construct
GYTVSSYCMG

SEQ ID NO: 63 - protein, 10 aa, Artificial Sequence
  Synthetic Construct
GYTVSSYCMG

SEQ ID NO: 64 - protein, 10 aa, Artificial Sequence
  Synthetic Construct
GYTVSSYCMG

SEQ ID NO: 65 - protein, 10 aa, Artificial Sequence
  Synthetic Construct
GYTVSSYCMG

SEQ ID NO: 66 - protein, 10 aa, Artificial Sequence
  Synthetic Construct
GYTVSSYCMG

SEQ ID NO: 67 - protein, 10 aa, Artificial Sequence
  Synthetic Construct
GYTVSSYCMG

SEQ ID NO: 68 - protein, 10 aa, Artificial Sequence
  Synthetic Construct
GYTVSSYCMG

SEQ ID NO: 69 - protein, 10 aa, Artificial Sequence
  Synthetic Construct
GYTVSSYCMG

SEQ ID NO: 70 - protein, 10 aa, Artificial Sequence
  Synthetic Construct
GYTVSSYCMG

SEQ ID NO: 71 - protein, 10 aa, Artificial Sequence
  Synthetic Construct
GYTYGGYCMG

SEQ ID NO: 72 - protein, 10 aa, Artificial Sequence
  Synthetic Construct
GYTYGGYCMG

SEQ ID NO: 73 - protein, 10 aa, Artificial Sequence
  Synthetic Construct
GYTYGGYCMG

SEQ ID NO: 74 - protein, 10 aa, Artificial Sequence
  Synthetic Construct
GYTYGGYCMG

SEQ ID NO: 75 - protein, 10 aa, Artificial Sequence
  Synthetic Construct
GYTYGGYCMG

SEQ ID NO: 76 - protein, 10 aa, Artificial Sequence
  Synthetic Construct
GYTYGGYCMG

SEQ ID NO: 77 - protein, 14 aa, Artificial Sequence
  Synthetic Construct
WFRQAPGKEREGVA

SEQ ID NO: 78 - protein, 14 aa, Artificial Sequence
  Synthetic Construct
WFRQAPGKEREGVA

SEQ ID NO: 79 - protein, 14 aa, Artificial Sequence
  Synthetic Construct
WFRQAPGKEREGVA

SEQ ID NO: 80 - protein, 14 aa, Artificial Sequence
  Synthetic Construct
WFRQAPGKEREGVA

SEQ ID NO: 81 - protein, 14 aa, Artificial Sequence
  Synthetic Construct
WFRQAPGKEREGVA

SEQ ID NO: 82 - protein, 14 aa, Artificial Sequence
  Synthetic Construct
WFRQAPGKEREGVS

SEQ ID NO: 83 - protein, 14 aa, Artificial Sequence
  Synthetic Construct
WFRQAPGKEREGVA

SEQ ID NO: 84 - protein, 14 aa, Artificial Sequence
  Synthetic Construct
WFRQAPGKEREGVA

SEQ ID NO: 85 - protein, 14 aa, Artificial Sequence
  Synthetic Construct
WFRQAPGKGLEGVS

SEQ ID NO: 86 - protein, 14 aa, Artificial Sequence
  Synthetic Construct
WFRQAPGKGLEGVA

SEQ ID NO: 87 - protein, 14 aa, Artificial Sequence
  Synthetic Construct
WFRQAPGKGLEGVA

SEQ ID NO: 88 - protein, 14 aa, Artificial Sequence
  Synthetic Construct
WFRQAPGKGREGVA

SEQ ID NO: 89 - protein, 14 aa, Artificial Sequence
  Synthetic Construct
WFRQAPGKEREGVA

SEQ ID NO: 90 - protein, 14 aa, Artificial Sequence
  Synthetic Construct
WFRQAPGKEREGVA

SEQ ID NO: 91 - protein, 14 aa, Artificial Sequence
  Synthetic Construct
WFRQAPGKGLEGVA

SEQ ID NO: 92 - protein, 14 aa, Artificial Sequence
  Synthetic Construct
WFRQAPGKGLEGVA

SEQ ID NO: 93 - protein, 14 aa, Artificial Sequence
  Synthetic Construct
WFRQAPGKGLEGVA

SEQ ID NO: 94 - protein, 14 aa, Artificial Sequence
  Synthetic Construct
WFRQAPGKGLEGVA

SEQ ID NO: 95 - protein, 14 aa, Artificial Sequence
  Synthetic Construct
WFRQAPGKGREGVA

SEQ ID NO: 96 - protein, 14 aa, Artificial Sequence
  Synthetic Construct
WFRQAPGKEREGVA

SEQ ID NO: 97 - protein, 14 aa, Artificial Sequence
  Synthetic Construct
WFRQAPGKEREGVA

SEQ ID NO: 98 - protein, 14 aa, Artificial Sequence
  Synthetic Construct
WFRQAPGKGLEGVA

SEQ ID NO: 99 - protein, 14 aa, Artificial Sequence
  Synthetic Construct
WFRQAPGKGLEGVA

SEQ ID NO: 100 - protein, 14 aa, Artificial Sequence
  Synthetic Construct
WFRQAPGKGLEGVS

SEQ ID NO: 101 - protein, 14 aa, Artificial Sequence
  Synthetic Construct
WFRQAPGKGLEGVS

SEQ ID NO: 102 - protein, 14 aa, Artificial Sequence
  Synthetic Construct
WFRQAPGKGLEGVA

SEQ ID NO: 103 - protein, 14 aa, Artificial Sequence
  Synthetic Construct
WFRQAPGKGLEGVA

SEQ ID NO: 104 - protein, 14 aa, Artificial Sequence
  Synthetic Construct
WFRQAPGKGREGVA

SEQ ID NO: 105 - protein, 14 aa, Artificial Sequence
  Synthetic Construct
WFRQAPGKEREGVA

SEQ ID NO: 106 - protein, 14 aa, Artificial Sequence
  Synthetic Construct
WFRQAPGKEREGVA

SEQ ID NO: 107 - protein, 14 aa, Artificial Sequence
  Synthetic Construct
WFRQAPGKGREGVS

SEQ ID NO: 108 - protein, 14 aa, Artificial Sequence
  Synthetic Construct
WFRQAPGKGREGVS

SEQ ID NO: 109 - protein, 14 aa, Artificial Sequence
  Synthetic Construct
WFRQAPGKGLEGVS

SEQ ID NO: 110 - protein, 14 aa, Artificial Sequence
  Synthetic Construct
WFRQAPGKGLEGVS

SEQ ID NO: 111 - protein, 14 aa, Artificial Sequence
  Synthetic Construct
WFRQAPGKGLEGVS

SEQ ID NO: 112 - protein, 14 aa, Artificial Sequence
  Synthetic Construct
WFRQAPGKGREGVS

SEQ ID NO: 113 - protein, 14 aa, Artificial Sequence
  Synthetic Construct
WFRQAPGKGREGVS

SEQ ID NO: 114 - protein, 14 aa, Artificial Sequence
  Synthetic Construct
WFRQAPGKGREGVS

SEQ ID NO: 115 - protein, 16 aa, Artificial Sequence
  Synthetic Construct
AIDSDGSTSYAGSVKG

SEQ ID NO: 116 - protein, 16 aa, Artificial Sequence
  Synthetic Construct
AIDSDGGTSYADSVKG

SEQ ID NO: 117 - protein, 16 aa, Artificial Sequence
  Synthetic Construct
AIDSDGSTSYADSVKG

SEQ ID NO: 118 - protein, 16 aa, Artificial Sequence
  Synthetic Construct
TINSDGSTNYADSVKG

SEQ ID NO: 119 - protein, 16 aa, Artificial Sequence
  Synthetic Construct
AIDSDGSVSYADSVKG

SEQ ID NO: 120 - protein, 17 aa, Artificial Sequence
  Synthetic Construct
CISWSGGSTYYTDSVKG

SEQ ID NO: 121 - protein, 16 aa, Artificial Sequence
  Synthetic Construct
AIDSDGSTSYADSVKG

SEQ ID NO: 122 - protein, 16 aa, Artificial Sequence
  Synthetic Construct
AIDSSGGTSYADSVKG

SEQ ID NO: 123 - protein, 16 aa, Artificial Sequence
  Synthetic Construct
AIDSDGGTSYADSVKG

SEQ ID NO: 124 - protein, 16 aa, Artificial Sequence
  Synthetic Construct
AIDSDGGTSYADSVKG

SEQ ID NO: 125 - protein, 16 aa, Artificial Sequence
  Synthetic Construct
AIDSDGGTSYADSVKG

SEQ ID NO: 126 - protein, 16 aa, Artificial Sequence
  Synthetic Construct
AIDSDGGTSYADSVKG

SEQ ID NO: 127 - protein, 16 aa, Artificial Sequence
  Synthetic Construct
AIDSDGGTSYADSVKG

SEQ ID NO: 128 - protein, 16 aa, Artificial Sequence
  Synthetic Construct
AIDSDGGTSYADSVKG

SEQ ID NO: 129 - protein, 16 aa, Artificial Sequence
  Synthetic Construct
AIDSDGGTSYADSVKG

SEQ ID NO: 130 - protein, 16 aa, Artificial Sequence
  Synthetic Construct
AIDSSGGTSYADSVKG

SEQ ID NO: 131 - protein, 16 aa, Artificial Sequence
  Synthetic Construct
AIDSDGSTSYADSVKG

SEQ ID NO: 132 - protein, 16 aa, Artificial Sequence
  Synthetic Construct
AIDSDGSTSYADSVKG

SEQ ID NO: 133 - protein, 16 aa, Artificial Sequence
  Synthetic Construct
AIDSDGSTSYADSVKG

SEQ ID NO: 134 - protein, 16 aa, Artificial Sequence
  Synthetic Construct
AIDSDGSTSYADSVKG

SEQ ID NO: 135 - protein, 16 aa, Artificial Sequence
  Synthetic Construct
AIDSDGSTSYADSVKG

SEQ ID NO: 136 - protein, 16 aa, Artificial Sequence
  Synthetic Construct
AIDSDGSTSYADSVKG

SEQ ID NO: 137 - protein, 16 aa, Artificial Sequence
  Synthetic Construct
AIDSSGSTSYADSVKG

SEQ ID NO: 138 - protein, 16 aa, Artificial Sequence
  Synthetic Construct
AIDSDGSVSYADSVKG

SEQ ID NO: 139 - protein, 16 aa, Artificial Sequence
  Synthetic Construct
AIDSDGSVSYADSVKG

SEQ ID NO: 140 - protein, 16 aa, Artificial Sequence
  Synthetic Construct
AIDSDGSVSYADSVKG

SEQ ID NO: 141 - protein, 16 aa, Artificial Sequence
  Synthetic Construct
AIDSDGSVSYADSVKG

SEQ ID NO: 142 - protein, 16 aa, Artificial Sequence
  Synthetic Construct
AIDSDGSVSYADSVKG

SEQ ID NO: 143 - protein, 16 aa, Artificial Sequence
  Synthetic Construct
AIDSDGSVSYADSVKG

SEQ ID NO: 144 - protein, 16 aa, Artificial Sequence
  Synthetic Construct
AIDSDGSVSYADSVKG

SEQ ID NO: 145 - protein, 16 aa, Artificial Sequence
  Synthetic Construct
AIDSDGSVSYADSVKG

SEQ ID NO: 146 - protein, 16 aa, Artificial Sequence
  Synthetic Construct
AIDSSGSVSYADSVKG

SEQ ID NO: 147 - protein, 16 aa, Artificial Sequence
  Synthetic Construct
TINSDGSTNYADSVKG

SEQ ID NO: 148 - protein, 16 aa, Artificial Sequence
  Synthetic Construct
TIASEGSTNYADSVKG

SEQ ID NO: 149 - protein, 16 aa, Artificial Sequence
  Synthetic Construct
TIASSGSTNYADSVKG

SEQ ID NO: 150 - protein, 16 aa, Artificial Sequence
  Synthetic Construct
TINSDGSTNYADSVKG

SEQ ID NO: 151 - protein, 16 aa, Artificial Sequence
  Synthetic Construct
TIASEGSTNYADSVKG

SEQ ID NO: 152 - protein, 16 aa, Artificial Sequence
  Synthetic Construct
TIASSGSTNYADSVKG

SEQ ID NO: 153 - protein, 32 aa, Artificial Sequence
  Synthetic Construct
RFTISKDNAENTLYLQMNSLKPEDTAMYYCAT

SEQ ID NO: 154 - protein, 32 aa, Artificial Sequence
  Synthetic Construct
RFTISKDNAKNTLYLQMDSLKPEDTAMYYCAA

SEQ ID NO: 155 - protein, 32 aa, Artificial Sequence
  Synthetic Construct
RFTISKDNAKNTLYLQMNSLKPEDTAMYYCAA

SEQ ID NO: 156 - protein, 32 aa, Artificial Sequence
  Synthetic Construct
RFTISKDNAKNTLYLQMNSLSPEDTAMYYCAV

SEQ ID NO: 157 - protein, 32 aa, Artificial Sequence
  Synthetic Construct
RFTISKDNAKNTLYLQMNSLKPEDTAMYFCAA

SEQ ID NO: 158 - protein, 32 aa, Artificial Sequence
  Synthetic Construct
RFTISRDNAKNTLYLQMNSLKPEDTAMYYCAA

SEQ ID NO: 159 - protein, 32 aa, Artificial Sequence
  Synthetic Construct
RFTISKDNAKNTLFLQMNGLKPEDTAVYYCAP

SEQ ID NO: 160 - protein, 32 aa, Artificial Sequence; identical to SEQ ID NO: 154
  Synthetic Construct

SEQ ID NO: 161 - protein, 32 aa, Artificial Sequence
  Synthetic Construct
RFTISRDNSKNTLYLQMNSLRAEDTAVYYCAA

SEQ ID NO: 162 - protein, 32 aa, Artificial Sequence; identical to SEQ ID NO: 161
  Synthetic Construct

SEQ ID NO: 163 - protein, 32 aa, Artificial Sequence
  Synthetic Construct
RFTISRDNSKNTLYLQMNSLRAEDTAMYYCAA

SEQ ID NO: 164 - protein, 32 aa, Artificial Sequence; identical to SEQ ID NO: 163
  Synthetic Construct

SEQ ID NO: 165 - protein, 32 aa, Artificial Sequence; identical to SEQ ID NO: 163
  Synthetic Construct

SEQ ID NO: 166 - protein, 32 aa, Artificial Sequence
  Synthetic Construct
RFTISKDNSKNTLYLQMNSLRAEDTAMYYCAA

SEQ ID NO: 167 - protein, 32 aa, Artificial Sequence; identical to SEQ ID NO: 166
  Synthetic Construct

SEQ ID NO: 168 - protein, 32 aa, Artificial Sequence; identical to SEQ ID NO: 166
  Synthetic Construct

SEQ ID NO: 169 - protein, 32 aa, Artificial Sequence; identical to SEQ ID NO: 161
  Synthetic Construct

SEQ ID NO: 170 - protein, 32 aa, Artificial Sequence; identical to SEQ ID NO: 163
  Synthetic Construct

SEQ ID NO: 171 - protein, 32 aa, Artificial Sequence; identical to SEQ ID NO: 163
  Synthetic Construct

SEQ ID NO: 172 - protein, 32 aa, Artificial Sequence; identical to SEQ ID NO: 163
  Synthetic Construct

SEQ ID NO: 173 - protein, 32 aa, Artificial Sequence; identical to SEQ ID NO: 166
  Synthetic Construct

SEQ ID NO: 174 - protein, 32 aa, Artificial Sequence
  Synthetic Construct
RFTISKDNSKNTLYLQMNSLRAEDTAVYYCAA

SEQ ID NO: 175 - protein, 32 aa, Artificial Sequence; identical to SEQ ID NO: 174
  Synthetic Construct

SEQ ID NO: 176 - protein, 32 aa, Artificial Sequence; identical to SEQ ID NO: 161
  Synthetic Construct

SEQ ID NO: 177 - protein, 32 aa, Artificial Sequence
  Synthetic Construct
RFTISRDNSKNTLYLQMNSLRAEDTAVYFCAA

SEQ ID NO: 178 - protein, 32 aa, Artificial Sequence; identical to SEQ ID NO: 177
  Synthetic Construct

SEQ ID NO: 179 - protein, 32 aa, Artificial Sequence
  Synthetic Construct
RFTISRDNSKNTLYLQMNSLRAEDTAMYFCAA

SEQ ID NO: 180 - protein, 32 aa, Artificial Sequence; identical to SEQ ID NO: 179
  Synthetic Construct

SEQ ID NO: 181 - protein, 32 aa, Artificial Sequence; identical to SEQ ID NO: 179
  Synthetic Construct

SEQ ID NO: 182 - protein, 32 aa, Artificial Sequence
  Synthetic Construct
RFTISKDNSKNTLYLQMNSLRAEDTAMYFCAA

SEQ ID NO: 183 - protein, 32 aa, Artificial Sequence
  Synthetic Construct
RFTISKDNSKNTLYLQMNSLRAEDTAVYFCAA

SEQ ID NO: 184 - protein, 32 aa, Artificial Sequence; identical to SEQ ID NO: 183
  Synthetic Construct

SEQ ID NO: 185 - protein, 32 aa, Artificial Sequence
  Synthetic Construct
RFTISRDNSKNTLYLQMNSLRAEDTAVYYCAV

SEQ ID NO: 186 - protein, 32 aa, Artificial Sequence; identical to SEQ ID NO: 185
  Synthetic Construct

SEQ ID NO: 187 - protein, 32 aa, Artificial Sequence; identical to SEQ ID NO: 185
  Synthetic Construct

SEQ ID NO: 188 - protein, 32 aa, Artificial Sequence
  Synthetic Construct
RFTISRDNAKNTLYLQMNSLRPEDTAVYYCAV

SEQ ID NO: 189 - protein, 32 aa, Artificial Sequence; identical to SEQ ID NO: 188
  Synthetic Construct

SEQ ID NO: 190 - protein, 32 aa, Artificial Sequence; identical to SEQ ID NO: 188
  Synthetic Construct

SEQ ID NO: 191 - protein, 16 aa, Artificial Sequence
  Synthetic Construct
SPLWLLSRLDPADFEY

SEQ ID NO: 192 - protein, 16 aa, Artificial Sequence
  Synthetic Construct
DFCWVDEDRHLYEYNS

SEQ ID NO: 193 - protein, 13 aa, Artificial Sequence
  Synthetic Construct
DFCWVDDFYEYNY

SEQ ID NO: 194 - protein, 18 aa, Artificial Sequence
  Synthetic Construct
DLAPCWVAGPIEAADFGY

SEQ ID NO: 195 - protein, 14 aa, Artificial Sequence
  Synthetic Construct
DLCWVDQDQGEYNT

SEQ ID NO: 196 - protein, 22 aa, Artificial Sequence
  Synthetic Construct
DLFCPPPDDTTGWGMDPPEHNY

SEQ ID NO: 197 - protein, 13 aa, Artificial Sequence
  Synthetic Construct
LCWVDYPLPSGPY

SEQ ID NO: 198 - protein, 16 aa, Artificial Sequence
  Synthetic Construct
DFCWVDEDRHLYEYQS

SEQ ID NO: 199 - protein, 16 aa, Artificial Sequence
  Synthetic Construct
DFCWVDEDRHLYEYNS

SEQ ID NO: 200 - protein, 16 aa, Artificial Sequence
  Synthetic Construct
DFCWVDEDRHLYEYNS

SEQ ID NO: 201 - protein, 16 aa, Artificial Sequence
  Synthetic Construct
DFCWVDEDRHLYEYNS

SEQ ID NO: 202 - protein, 16 aa, Artificial Sequence
  Synthetic Construct
DFCWVDEDRHLYEYNS

SEQ ID NO: 203 - protein, 16 aa, Artificial Sequence
  Synthetic Construct
DFCWVDEDRHLYEYNS

SEQ ID NO: 204 - protein, 16 aa, Artificial Sequence
  Synthetic Construct
DFCWVDEDRHLYEYNS

SEQ ID NO: 205 - protein, 16 aa, Artificial Sequence
  Synthetic Construct
DFCWVDEDRHLYEYNS

SEQ ID NO: 206 - protein, 16 aa, Artificial Sequence
  Synthetic Construct
DFCWVDEDRHLYEYNS

SEQ ID NO: 207 - protein, 13 aa, Artificial Sequence
  Synthetic Construct
DFCWVDDFYEYNY

SEQ ID NO: 208 - protein, 13 aa, Artificial Sequence
  Synthetic Construct
DFCWVDDFYEYNY

SEQ ID NO: 209 - protein, 13 aa, Artificial Sequence
  Synthetic Construct
DFCWVDDFYEYNY

SEQ ID NO: 210 - protein, 13 aa, Artificial Sequence
  Synthetic Construct
DFCWVDDFYEYNY

SEQ ID NO: 211 - protein, 13 aa, Artificial Sequence
  Synthetic Construct
DFCWVDDFYEYNY

SEQ ID NO: 212 - protein, 13 aa, Artificial Sequence
  Synthetic Construct
DFCWVDDFYEYNY

SEQ ID NO: 213 - protein, 13 aa, Artificial Sequence
  Synthetic Construct
DFCWVDDFYEYNY

SEQ ID NO: 214 - protein, 14 aa, Artificial Sequence
  Synthetic Construct
DLCWVDQDQGEYNT

SEQ ID NO: 215 - protein, 14 aa, Artificial Sequence
  Synthetic Construct
DLCWVDQDQGEYNT

SEQ ID NO: 216 - protein, 14 aa, Artificial Sequence
  Synthetic Construct
DLCWVDQDQGEYNT

SEQ ID NO: 217 - protein, 14 aa, Artificial Sequence
  Synthetic Construct
DLCWVDQDQGEYNT

SEQ ID NO: 218 - protein, 14 aa, Artificial Sequence
  Synthetic Construct
DLCWVDQDQGEYNT

SEQ ID NO: 219 - protein, 14 aa, Artificial Sequence
  Synthetic Construct
DLCWVDQDQGEYNT

SEQ ID NO: 220 - protein, 14 aa, Artificial Sequence
  Synthetic Construct
DLCWVDQDQGEYNT

SEQ ID NO: 221 - protein, 14 aa, Artificial Sequence
  Synthetic Construct
DLCWVDQDQGEYNT

SEQ ID NO: 222 - protein, 14 aa, Artificial Sequence
  Synthetic Construct
DLCWVDQDQGEYNT

SEQ ID NO: 223 - protein, 18 aa, Artificial Sequence
  Synthetic Construct
DLAPCWVAGPIEAADFGY

SEQ ID NO: 224 - protein, 18 aa, Artificial Sequence
  Synthetic Construct
DLAPCWVAGPIEAADFGY

SEQ ID NO: 225 - protein, 18 aa, Artificial Sequence
  Synthetic Construct
DLAPCWVAGPIEAADFGY

SEQ ID NO: 226 - protein, 18 aa, Artificial Sequence
  Synthetic Construct
DLAPCWVAGPIEAADFGY

SEQ ID NO: 227 - protein, 18 aa, Artificial Sequence
  Synthetic Construct
DLAPCWVAGPIEAADFGY

SEQ ID NO: 228 - protein, 18 aa, Artificial Sequence
  Synthetic Construct
DLAPCWVAGPIEAADFGY

SEQ ID NO: 229 - protein, 11 aa, Artificial Sequence
  Synthetic Construct
WGQGTQVTVSS

SEQ ID NO: 230 - protein, 11 aa, Artificial Sequence
  Synthetic Construct
WGQGTQVTVSS

SEQ ID NO: 231 - protein, 11 aa, Artificial Sequence
  Synthetic Construct
WGQGTQVTVSS

SEQ ID NO: 232 - protein, 11 aa, Artificial Sequence
  Synthetic Construct
WGQGTQVTVSS

SEQ ID NO: 233 - protein, 11 aa, Artificial Sequence
  Synthetic Construct
WGQGTQVTVSS

SEQ ID NO: 234 - protein, 11 aa, Artificial Sequence
  Synthetic Construct
WGQGTQVTVSS

SEQ ID NO: 235 - protein, 11 aa, Artificial Sequence
  Synthetic Construct
WGQGTQVTVSS

SEQ ID NO: 236 - protein, 11 aa, Artificial Sequence
  Synthetic Construct
WGQGTQVTVSS

SEQ ID NO: 237 - protein, 11 aa, Artificial Sequence
  Synthetic Construct
WGQGTLVTVSS

SEQ ID NO: 238 - protein, 11 aa, Artificial Sequence
  Synthetic Construct
WGQGTLVTVSS

SEQ ID NO: 239 - protein, 11 aa, Artificial Sequence
  Synthetic Construct
WGQGTLVTVSS

SEQ ID NO: 240 - protein, 11 aa, Artificial Sequence
  Synthetic Construct
WGQGTLVTVSS

SEQ ID NO: 241 - protein, 11 aa, Artificial Sequence
  Synthetic Construct
WGQGTLVTVSS

SEQ ID NO: 242 - protein, 11 aa, Artificial Sequence
  Synthetic Construct
WGQGTLVTVSS

SEQ ID NO: 243 - protein, 11 aa, Artificial Sequence
  Synthetic Construct
WGQGTLVTVSS

SEQ ID NO: 244 - protein, 11 aa, Artificial Sequence
  Synthetic Construct
WGQGTLVTVSS

SEQ ID NO: 245 - protein, 11 aa, Artificial Sequence
  Synthetic Construct
WGQGTLVTVSS

SEQ ID NO: 246 - protein, 11 aa, Artificial Sequence
  Synthetic Construct
WGQGTLVTVSS

SEQ ID NO: 247 - protein, 11 aa, Artificial Sequence
  Synthetic Construct
WGQGTLVTVSS

SEQ ID NO: 248 - protein, 11 aa, Artificial Sequence
  Synthetic Construct
WGQGTLVTVSS

SEQ ID NO: 249 - protein, 11 aa, Artificial Sequence
  Synthetic Construct
WGQGTLVTVSS

SEQ ID NO: 250 - protein, 11 aa, Artificial Sequence
  Synthetic Construct
WGQGTLVTVSS

SEQ ID NO: 251 - protein, 11 aa, Artificial Sequence
  Synthetic Construct
WGQGTLVTVSS

SEQ ID NO: 252 - protein, 11 aa, Artificial Sequence
  Synthetic Construct
WGQGTLVTVSS

SEQ ID NO: 253 - protein, 11 aa, Artificial Sequence
  Synthetic Construct
WGQGTLVTVSS

SEQ ID NO: 254 - protein, 11 aa, Artificial Sequence
  Synthetic Construct
WGQGTLVTVSS

SEQ ID NO: 255 - protein, 11 aa, Artificial Sequence
  Synthetic Construct
WGQGTLVTVSS

SEQ ID NO: 256 - protein, 11 aa, Artificial Sequence
  Synthetic Construct
WGQGTLVTVSS

SEQ ID NO: 257 - protein, 11 aa, Artificial Sequence
  Synthetic Construct
WGQGTLVTVSS

SEQ ID NO: 258 - protein, 11 aa, Artificial Sequence
  Synthetic Construct
WGQGTLVTVSS

SEQ ID NO: 259 - protein, 11 aa, Artificial Sequence
  Synthetic Construct
WGQGTLVTVSS

SEQ ID NO: 260 - protein, 11 aa, Artificial Sequence
  Synthetic Construct
WGQGTLVTVSS

SEQ ID NO: 261 - protein, 11 aa, Artificial Sequence
  Synthetic Construct
WGQGTLVTVSS

SEQ ID NO: 262 - protein, 11 aa, Artificial Sequence
  Synthetic Construct
WGQGTLVTVSS

SEQ ID NO: 263 - protein, 11 aa, Artificial Sequence
  Synthetic Construct
WGQGTLVTVSS

SEQ ID NO: 264 - protein, 11 aa, Artificial Sequence
  Synthetic Construct
WGQGTLVTVSS

SEQ ID NO: 265 - protein, 11 aa, Artificial Sequence
  Synthetic Construct
WGQGTLVTVSS

SEQ ID NO: 266 - protein, 11 aa, Artificial Sequence
  Synthetic Construct
WGQGTLVTVSS

SEQ ID NO: 267 - DNA, 372 bp, Artificial Sequence
  Synthetic Construct
caggtgcaactggcggagtctgggggaggctcggtgcatgctggagggtctctgagactctcctgtgtagtttctgaatataccttcagtagtgattctatgggctggttccgccaggctccagggaaggagcgcgagggggtcgcagctattgatagtgatggtagcacaagctacgcaggctccgtgaaggggcgattcaccatctccaaagacaacgccgagaacactctgtatctgcaaatgaacagcctgaaacctgaggacactgccatgtactactgtgcgacaagccctctgtggctgctatccaggctcgacccagctgactttgaatactggggccaggggacccaggtcaccgtctcctca

SEQ ID NO: 268 - DNA, 372 bp, Artificial Sequence
  Synthetic Construct
gaggtgcaactggtggagtctgggggaggctcggtgcaggctggagggtctctgagactctcctgtgcagcctctggatacatcatcagtagctactgcatgggctggttccgccaggctccagggaaggagcgcgagggggtcgcagctattgatagtgatggtggcacaagctacgcagactccgtgaagggccgattcaccatctccaaagacaacgccaagaacactctgtatctgcaaatggacagcctgaaacctgaggacactgccatgtactactgtgcggcagatttttgttgggtagatgaggatcgccacctctatgagtataactcctggggccaggggacccaggtcaccgtctcctca

SEQ ID NO: 269 - DNA, 363 bp, Artificial Sequence
  Synthetic Construct
caggtgcagctggcggagtctgggggaggctcggtgcaggctggagggtctctgagactctcctgtgcagcctctggatacaccatcagtagctactgcatgggctggttccgccaggctccagggaaggagcgcgagggggtcgcagctattgatagtgatggtagcacaagctacgcagactccgtgaagggccgattcaccatctccaaagacaacgccaagaacactctgtatctgcaaatgaacagcctgaaacctgaggacactgccatgtactactgtgcggcagatttttgttgggtggacgacttctatgagtataactactggggccaggggacccaggtcaccgtctcctca

SEQ ID NO: 270 - DNA, 378 bp, Artificial Sequence
  Synthetic Construct
gaggtgcaactggcggagtctgggggaggctcggtgcaggctggagggtctctgagactctcctgtgcagcctctggatacacctacggtggctactgcatgggctggttccgccaggctccagggaaggagcgcgagggggtcgcaactattaatagtgatggtagcacaaactacgcagactccgtgaagggccgattcaccatctccaaagacaacgccaagaacactctgtatctgcaaatgaacagcctgagccctgaggacactgccatgtactactgcgcggtggatctcgccccatgttgggtagctggtcccatcgaggccgctgactttggttactggggccaggggacccaggtcaccgtctcctca

SEQ ID NO: 271 - DNA, 366 bp, Artificial Sequence
  Synthetic Construct
caggtgcacctgatggagtctgggggaggctcggtgcaggttggagggtctctgagactctcctgtgcagcctctggatacaccgtcagtagctactgcatgggctggttccgccaggctccagggaaggagcgcgagggggtcgcagctattgatagtgatggtagcgtaagttatgcagactccgtgaagggccgattcaccatctccaaagacaacgccaagaacactctgtatctgcaaatgaacagcctgaaacctgaggacactgccatgtacttctgtgcggcagatctttgctgggtggaccaggaccagggagaatataacacctggggccaggggacccaggtcaccgtctcctca

SEQ ID NO: 272 - DNA, 393 bp, Artificial Sequence
  Synthetic Construct
gaggtgcagctggtggagtctgggggaggcttggtgcaggcaggggggtctctgagactctcctgtacagcctctggattgacttttgatgattatgccatgggctggttccgccaggctccagggaaggagcgcgagggggtctcatgtattagctggagtggtggtagcacatactataccgactccgtgaagggccgattcaccatctccagagacaacgccaagaacacgctgtatctgcaaatgaacagcctgaaacctgaggacacggccatgtattactgtgcggcagatttgttctgtcccccacctgatgatactacgggttggggtatggaccctcccgagcataactactggggccaggggacccaggtcaccgtctcctca

SEQ ID NO: 273 - DNA, 363 bp, Artificial Sequence
  Synthetic Construct
caggttcagctggtggagtctgggggaggctcggtgcaggctggagggtctctgagactttcctgtgcagcctctggatacaccttgagtagctactgcatgggctggttccgccaggctccagggaaggagcgcgagggggtcgcagctattgatagtgatggtagcacaagctacgcagactccgtgaagggccgattcaccatctccaaagacaacgccaagaacactctgtttctgcaaatgaacggcctgaaacctgaggacactgcggtgtactactgtgctccactatgctgggttgattacccattgccgtcgggcccatactggggccaggggacccaggtcaccgtctcctca

SEQ ID NO: 274 - protein, 124 aa, Artificial Sequence
  Synthetic Construct
QVQLAESGGGSVHAGGSLRLSCVVSEYTFSSDSMGWFRQAPGKEREGVAAIDSDGSTSYAGSVKGRFTISKDNAENTLYLQMNSLKPEDTAMYYCATSPLWLLSRLDPADFEYWGQGTQVTVSS

SEQ ID NO: 275 - protein, 124 aa, Artificial Sequence
  Synthetic Construct
EVQLVESGGGSVQAGGSLRLSCAASGYIISSYCMGWFRQAPGKEREGVAAIDSDGGTSYADSVKGRFTISKDNAKNTLYLQMDSLKPEDTAMYYCAADFCWVDEDRHLYEYNSWGQGTQVTVSS

SEQ ID NO: 276 - protein, 121 aa, Artificial Sequence
  Synthetic Construct
QVQLAESGGGSVQAGGSLRLSCAASGYTISSYCMGWFRQAPGKEREGVAAIDSDGSTSYADSVKGRFTISKDNAKNTLYLQMNSLKPEDTAMYYCAADFCWVDDFYEYNYWGQGTQVTVSS

SEQ ID NO: 277 - protein, 126 aa, Artificial Sequence
  Synthetic Construct
EVQLAESGGGSVQAGGSLRLSCAASGYTYGGYCMGWFRQAPGKEREGVATINSDGSTNYADSVKGRFTISKDNAKNTLYLQMNSLSPEDTAMYYCAVDLAPCWVAGPIEAADFGYWGQGTQVTVSS

SEQ ID NO: 278 - protein, 122 aa, Artificial Sequence
  Synthetic Construct
QVHLMESGGGSVQVGGSLRLSCAASGYTVSSYCMGWFRQAPGKEREGVAAIDSDGSVSYADSVKGRFTISKDNAKNTLYLQMNSLKPEDTAMYFCAADLCWVDQDQGEYNTWGQGTQVTVSS

SEQ ID NO: 279 - protein, 131 aa, Artificial Sequence
  Synthetic Construct
EVQLVESGGGLVQAGGSLRLSCTASGLTFDDYAMGWFRQAPGKEREGVSCISWSGGSTYYTDSVKGRFTISRDNAKNTLYLQMNSLKPEDTAMYYCAADLFCPPPDDTTGWGMDPPEHNYWGQGTQVTVSS

SEQ ID NO: 280 - protein, 121 aa, Artificial Sequence
  Synthetic Construct
QVQLVESGGGSVQAGGSLRLSCAASGYTLSSYCMGWFRQAPGKEREGVAAIDSDGSTSYADSVKGRFTISKDNAKNTLFLQMNGLKPEDTAVYYCAPLCWVDYPLPSGPYWGQGTQVTVSS

SEQ ID NO: 281 - protein, 124 aa, Artificial Sequence
  Synthetic Construct
EVQLVESGGGSVQAGGSLRLSCAASGYIISSYCMGWFRQAPGKEREGVAAIDSSGGTSYADSVKGRFTISKDNAKNTLYLQMDSLKPEDTAMYYCAADFCWVDEDRHLYEYQSWGQGTQVTVSS

SEQ ID NO: 282 - protein, 124 aa, Artificial Sequence
  Synthetic Construct
EVQLVESGGGLVQPGGSLRLSCAASGYIISSYCMGWFRQAPGKGLEGVSAIDSDGGTSYADSVKGRFTISRDNSKNTLYLQMNSLRAEDTAVYYCAADFCWVDEDRHLYEYNSWGQGTLVTVSS

SEQ ID NO: 283 - protein, 124 aa, Artificial Sequence
  Synthetic Construct
EVQLVESGGGLVQPGGSLRLSCAASGYIISSYCMGWFRQAPGKGLEGVAAIDSDGGTSYADSVKGRFTISRDNSKNTLYLQMNSLRAEDTAVYYCAADFCWVDEDRHLYEYNSWGQGTLVTVSS

SEQ ID NO: 284 - protein, 124 aa, Artificial Sequence
  Synthetic Construct
EVQLVESGGGLVQPGGSLRLSCAASGYIISSYCMGWFRQAPGKGLEGVAAIDSDGGTSYADSVKGRFTISRDNSKNTLYLQMNSLRAEDTAMYYCAADFCWVDEDRHLYEYNSWGQGTLVTVSS

SEQ ID NO: 285 - protein, 124 aa, Artificial Sequence
  Synthetic Construct
EVQLVESGGGLVQPGGSLRLSCAASGYIISSYCMGWFRQAPGKGREGVAAIDSDGGTSYADSVKGRFTISRDNSKNTLYLQMNSLRAEDTAMYYCAADFCWVDEDRHLYEYNSWGQGTLVTVSS

SEQ ID NO: 286 - protein, 124 aa, Artificial Sequence
  Synthetic Construct
EVQLVESGGGLVQPGGSLRLSCAASGYIISSYCMGWFRQAPGKEREGVAAIDSDGGTSYADSVKGRFTISRDNSKNTLYLQMNSLRAEDTAMYYCAADFCWVDEDRHLYEYNSWGQGTLVTVSS

SEQ ID NO: 287 - protein, 124 aa, Artificial Sequence
  Synthetic Construct
EVQLVESGGGLVQPGGSLRLSCAASGYIISSYCMGWFRQAPGKEREGVAAIDSDGGTSYADSVKGRFTISKDNSKNTLYLQMNSLRAEDTAMYYCAADFCWVDEDRHLYEYNSWGQGTLVTVSS

SEQ ID NO: 288 - protein, 124 aa, Artificial Sequence
  Synthetic Construct
EVQLVESGGGLVQPGGSLRLSCAASGYIISSYCMGWFRQAPGKGLEGVAAIDSDGGTSYADSVKGRFTISKDNSKNTLYLQMNSLRAEDTAMYYCAADFCWVDEDRHLYEYNSWGQGTLVTVSS

SEQ ID NO: 289 - protein, 124 aa, Artificial Sequence
  Synthetic Construct
EVQLVESGGGLVQPGGSLRLSCAASGYIISSYCMGWFRQAPGKGLEGVAAIDSSGGTSYADSVKGRFTISKDNSKNTLYLQMNSLRAEDTAMYYCAADFCWVDEDRHLYEYNSWGQGTLVTVSS

SEQ ID NO: 290 - protein, 121 aa, Artificial Sequence
  Synthetic Construct
EVQLVESGGGLVQPGGSLRLSCAASGYTISSYCMGWFRQAPGKGLEGVAAIDSDGSTSYADSVKGRFTISRDNSKNTLYLQMNSLRAEDTAVYYCAADFCWVDDFYEYNYWGQGTLVTVSS

SEQ ID NO: 291 - protein, 121 aa, Artificial Sequence
  Synthetic Construct
EVQLVESGGGLVQPGGSLRLSCAASGYTISSYCMGWFRQAPGKGLEGVAAIDSDGSTSYADSVKGRFTISRDNSKNTLYLQMNSLRAEDTAMYYCAADFCWVDDFYEYNYWGQGTLVTVSS

SEQ ID NO: 292 - protein, 121 aa, Artificial Sequence
  Synthetic Construct
EVQLVESGGGLVQPGGSLRLSCAASGYTISSYCMGWFRQAPGKGREGVAAIDSDGSTSYADSVKGRFTISRDNSKNTLYLQMNSLRAEDTAMYYCAADFCWVDDFYEYNYWGQGTLVTVSS

SEQ ID NO: 293 - protein, 121 aa, Artificial Sequence
  Synthetic Construct
EVQLVESGGGLVQPGGSLRLSCAASGYTISSYCMGWFRQAPGKEREGVAAIDSDGSTSYADSVKGRFTISRDNSKNTLYLQMNSLRAEDTAMYYCAADFCWVDDFYEYNYWGQGTLVTVSS

SEQ ID NO: 294 - protein, 121 aa, Artificial Sequence
  Synthetic Construct
EVQLVESGGGLVQPGGSLRLSCAASGYTISSYCMGWFRQAPGKEREGVAAIDSDGSTSYADSVKGRFTISKDNSKNTLYLQMNSLRAEDTAMYYCAADFCWVDDFYEYNYWGQGTLVTVSS

SEQ ID NO: 295 - protein, 121 aa, Artificial Sequence
  Synthetic Construct
EVQLVESGGGLVQPGGSLRLSCAASGYTISSYCMGWFRQAPGKGLEGVAAIDSDGSTSYADSVKGRFTISKDNSKNTLYLQMNSLRAEDTAVYYCAADFCWVDDFYEYNYWGQGTLVTVSS

SEQ ID NO: 296 - protein, 121 aa, Artificial Sequence
  Synthetic Construct
EVQLVESGGGLVQPGGSLRLSCAASGYTISSYCMGWFRQAPGKGLEGVAAIDSSGSTSYADSVKGRFTISKDNSKNTLYLQMNSLRAEDTAVYYCAADFCWVDDFYEYNYWGQGTLVTVSS

SEQ ID NO: 297 - protein, 122 aa, Artificial Sequence
  Synthetic Construct
EVQLVESGGGLVQPGGSLRLSCAASGYTVSSYCMGWFRQAPGKGLEGVSAIDSDGSVSYADSVKGRFTISRDNSKNTLYLQMNSLRAEDTAVYYCAADLCWVDQDQGEYNTWGQGTLVTVSS

SEQ ID NO: 298 - protein, 122 aa, Artificial Sequence
  Synthetic Construct
EVQLVESGGGLVQPGGSLRLSCAASGYTVSSYCMGWFRQAPGKGLEGVSAIDSDGSVSYADSVKGRFTISRDNSKNTLYLQMNSLRAEDTAVYFCAADLCWVDQDQGEYNTWGQGTLVTVSS

SEQ ID NO: 299 - protein, 122 aa, Artificial Sequence
  Synthetic Construct
EVQLVESGGGLVQPGGSLRLSCAASGYTVSSYCMGWFRQAPGKGLEGVAAIDSDGSVSYADSVKGRFTISRDNSKNTLYLQMNSLRAEDTAVYFCAADLCWVDQDQGEYNTWGQGTLVTVSS

SEQ ID NO: 300 - protein, 122 aa, Artificial Sequence
  Synthetic Construct
EVQLVESGGGLVQPGGSLRLSCAASGYTVSSYCMGWFRQAPGKGLEGVAAIDSDGSVSYADSVKGRFTISRDNSKNTLYLQMNSLRAEDTAMYFCAADLCWVDQDQGEYNTWGQGTLVTVSS

SEQ ID NO: 301 - protein, 122 aa, Artificial Sequence
  Synthetic Construct
EVQLVESGGGLVQPGGSLRLSCAASGYTVSSYCMGWFRQAPGKGREGVAAIDSDGSVSYADSVKGRFTISRDNSKNTLYLQMNSLRAEDTAMYFCAADLCWVDQDQGEYNTWGQGTLVTVSS

SEQ ID NO: 302 - protein, 122 aa, Artificial Sequence
  Synthetic Construct
EVQLVESGGGLVQPGGSLRLSCAASGYTVSSYCMGWFRQAPGKEREGVAAIDSDGSVSYADSVKGRFTISRDNSKNTLYLQMNSLRAEDTAMYFCAADLCWVDQDQGEYNTWGQGTLVTVSS

SEQ ID NO: 303 - protein, 122 aa, Artificial Sequence
  Synthetic Construct
EVQLVESGGGLVQPGGSLRLSCAASGYTVSSYCMGWFRQAPGKEREGVAAIDSDGSVSYADSVKGRFTISKDNSKNTLYLQMNSLRAEDTAMYFCAADLCWVDQDQGEYNTWGQGTLVTVSS

SEQ ID NO: 304 - protein, 122 aa, Artificial Sequence
  Synthetic Construct
EVQLVESGGGLVQPGGSLRLSCAASGYTVSSYCMGWFRQAPGKGREGVSAIDSDGSVSYADSVKGRFTISKDNSKNTLYLQMNSLRAEDTAVYFCAADLCWVDQDQGEYNTWGQGTLVTVSS

SEQ ID NO: 305 - protein, 122 aa, Artificial Sequence
  Synthetic Construct
EVQLVESGGGLVQPGGSLRLSCAASGYTVSSYCMGWFRQAPGKGREGVSAIDSSGSVSYADSVKGRFTISKDNSKNTLYLQMNSLRAEDTAVYFCAADLCWVDQDQGEYNTWGQGTLVTVSS

SEQ ID NO: 306 - protein, 126 aa, Artificial Sequence
  Synthetic Construct
EVQLVESGGGLVQPGGSLRLSCAASGYTYGGYCMGWFRQAPGKGLEGVSTINSDGSTNYADSVKGRFTISRDNSKNTLYLQMNSLRAEDTAVYYCAVDLAPCWVAGPIEAADFGYWGQGTLVTVSS

SEQ ID NO: 307 - protein, 126 aa, Artificial Sequence
  Synthetic Construct
EVQLVESGGGLVQPGGSLRLSCAASGYTYGGYCMGWFRQAPGKGLEGVSTIASEGSTNYADSVKGRFTISRDNSKNTLYLQMNSLRAEDTAVYYCAVDLAPCWVAGPIEAADFGYWGQGTLVTVSS

SEQ ID NO: 308 - protein, 126 aa, Artificial Sequence
  Synthetic Construct
EVQLVESGGGLVQPGGSLRLSCAASGYTYGGYCMGWFRQAPGKGLEGVSTIASSGSTNYADSVKGRFTISRDNSKNTLYLQMNSLRAEDTAVYYCAVDLAPCWVAGPIEAADFGYWGQGTLVTVSS

SEQ ID NO: 309 - protein, 126 aa, Artificial Sequence
  Synthetic Construct
EVQLVESGGGLVQPGGSLRLSCAASGYTYGGYCMGWFRQAPGKGREGVSTINSDGSTNYADSVKGRFTISRDNAKNTLYLQMNSLRPEDTAVYYCAVDLAPCWVAGPIEAADFGYWGQGTLVTVSS

SEQ ID NO: 310 - protein, 126 aa, Artificial Sequence
  Synthetic Construct
EVQLVESGGGLVQPGGSLRLSCAASGYTYGGYCMGWFRQAPGKGREGVSTIASEGSTNYADSVKGRFTISRDNAKNTLYLQMNSLRPEDTAVYYCAVDLAPCWVAGPIEAADFGYWGQGTLVTVSS

SEQ ID NO: 311 - protein, 126 aa, Artificial Sequence
  Synthetic Construct
EVQLVESGGGLVQPGGSLRLSCAASGYTYGGYCMGWFRQAPGKGREGVSTIASSGSTNYADSVKGRFTISRDNAKNTLYLQMNSLRPEDTAVYYCAVDLAPCWVAGPIEAADFGYWGQGTLVTVSS

SEQ ID NO: 312 - protein, 353 aa, Artificial Sequence
  Synthetic Construct
QVQLAESGGGSVHAGGSLRLSCVVSEYTFSSDSMGWFRQAPGKEREGVAAIDSDGSTSYAGSVKGRFTISKDNAENTLYLQMNSLKPEDTAMYYCATSPLWLLSRLDPADFEYWGQGTQVTVSSESKYGPPCPPCPAPEFLGGPSVFLFPPKPKDTLMISRTPEVTCVVVDVSQEDPEVQFNWYVDGVEVHNAKTKPREEQFNSTYRVVSVLTVLHQDWLNGKEYKCKVSNKGLPSSIEKTISKAKGQPREPQVYTLPPSQEEMTKNQVSLTCLVKGFYPSDIAVEWESNGQPENNYKTTPPVLDSDGSFFLYSRLTVDKSRWQEGNVFSCSVMHEALHNHYTQKSLSLSLGK

SEQ ID NO: 313 - protein, 353 aa, Artificial Sequence
  Synthetic Construct
EVQLVESGGGSVQAGGSLRLSCAASGYIISSYCMGWFRQAPGKEREGVAAIDSDGGTSYADSVKGRFTISKDNAKNTLYLQMDSLKPEDTAMYYCAADFCWVDEDRHLYEYNSWGQGTQVTVSSESKYGPPCPPCPAPEFLGGPSVFLFPPKPKDTLMISRTPEVTCVVVDVSQEDPEVQFNWYVDGVEVHNAKTKPREEQFNSTYRVVSVLTVLHQDWLNGKEYKCKVSNKGLPSSIEKTISKAKGQPREPQVYTLPPSQEEMTKNQVSLTCLVKGFYPSDIAVEWESNGQPENNYKTTPPVLDSDGSFFLYSRLTVDKSRWQEGNVFSCSVMHEALHNHYTQKSLSLSLGK

SEQ ID NO: 314 - protein, 350 aa, Artificial Sequence
  Synthetic Construct
QVQLAESGGGSVQAGGSLRLSCAASGYTISSYCMGWFRQAPGKEREGVAAIDSDGSTSYADSVKGRFTISKDNAKNTLYLQMNSLKPEDTAMYYCAADFCWVDDFYEYNYWGQGTQVTVSSESKYGPPCPPCPAPEFLGGPSVFLFPPKPKDTLMISRTPEVTCVVVDVSQEDPEVQFNWYVDGVEVHNAKTKPREEQFNSTYRVVSVLTVLHQDWLNGKEYKCKVSNKGLPSSIEKTISKAKGQPREPQVYTLPPSQEEMTKNQVSLTCLVKGFYPSDIAVEWESNGQPENNYKTTPPVLDSDGSFFLYSRLTVDKSRWQEGNVFSCSVMHEALHNHYTQKSLSLSLGK

SEQ ID NO: 315 - protein, 355 aa, Artificial Sequence
  Synthetic Construct
EVQLAESGGGSVQAGGSLRLSCAASGYTYGGYCMGWFRQAPGKEREGVATINSDGSTNYADSVKGRFTISKDNAKNTLYLQMNSLSPEDTAMYYCAVDLAPCWVAGPIEAADFGYWGQGTQVTVSSESKYGPPCPPCPAPEFLGGPSVFLFPPKPKDTLMISRTPEVTCVVVDVSQEDPEVQFNWYVDGVEVHNAKTKPREEQFNSTYRVVSVLTVLHQDWLNGKEYKCKVSNKGLPSSIEKTISKAKGQPREPQVYTLPPSQEEMTKNQVSLTCLVKGFYPSDIAVEWESNGQPENNYKTTPPVLDSDGSFFLYSRLTVDKSRWQEGNVFSCSVMHEALHNHYTQKSLSLSLGK

SEQ ID NO: 316 - protein, 351 aa, Artificial Sequence
  Synthetic Construct
QVHLMESGGGSVQVGGSLRLSCAASGYTVSSYCMGWFRQAPGKEREGVAAIDSDGSVSYADSVKGRFTISKDNAKNTLYLQMNSLKPEDTAMYFCAADLCWVDQDQGEYNTWGQGTQVTVSSESKYGPPCPPCPAPEFLGGPSVFLFPPKPKDTLMISRTPEVTCVVVDVSQEDPEVQFNWYVDGVEVHNAKTKPREEQFNSTYRVVSVLTVLHQDWLNGKEYKCKVSNKGLPSSIEKTISKAKGQPREPQVYTLPPSQEEMTKNQVSLTCLVKGFYPSDIAVEWESNGQPENNYKTTPPVLDSDGSFFLYSRLTVDKSRWQEGNVFSCSVMHEALHNHYTQKSLSLSLGK

SEQ ID NO: 317 - protein, 360 aa, Artificial Sequence
  Synthetic Construct
EVQLVESGGGLVQAGGSLRLSCTASGLTFDDYAMGWFRQAPGKEREGVSCISWSGGSTYYTDSVKGRFTISRDNAKNTLYLQMNSLKPEDTAMYYCAADLFCPPPDDTTGWGMDPPEHNYWGQGTQVTVSSESKYGPPCPPCPAPEFLGGPSVFLFPPKPKDTLMISRTPEVTCVVVDVSQEDPEVQFNWYVDGVEVHNAKTKPREEQFNSTYRVVSVLTVLHQDWLNGKEYKCKVSNKGLPSSIEKTISKAKGQPREPQVYTLPPSQEEMTKNQVSLTCLVKGFYPSDIAVEWESNGQPENNYKTTPPVLDSDGSFFLYSRLTVDKSRWQEGNVFSCSVMHEALHNHYTQKSLSLSLGK

SEQ ID NO: 318 - protein, 350 aa, Artificial Sequence
  Synthetic Construct
QVQLVESGGGSVQAGGSLRLSCAASGYTLSSYCMGWFRQAPGKEREGVAAIDSDGSTSYADSVKGRFTISKDNAKNTLFLQMNGLKPEDTAVYYCAPLCWVDYPLPSGPYWGQGTQVTVSSESKYGPPCPPCPAPEFLGGPSVFLFPPKPKDTLMISRTPEVTCVVVDVSQEDPEVQFNWYVDGVEVHNAKTKPREEQFNSTYRVVSVLTVLHQDWLNGKEYKCKVSNKGLPSSIEKTISKAKGQPREPQVYTLPPSQEEMTKNQVSLTCLVKGFYPSDIAVEWESNGQPENNYKTTPPVLDSDGSFFLYSRLTVDKSRWQEGNVFSCSVMHEALHNHYTQKSLSLSLGK

SEQ ID NO: 319 - protein, 353 aa, Artificial Sequence
  Synthetic Construct
EVQLVESGGGSVQAGGSLRLSCAASGYIISSYCMGWFRQAPGKEREGVAAIDSSGGTSYADSVKGRFTISKDNAKNTLYLQMDSLKPEDTAMYYCAADFCWVDEDRHLYEYQSWGQGTQVTVSSESKYGPPCPPCPAPEFLGGPSVFLFPPKPKDTLMISRTPEVTCVVVDVSQEDPEVQFNWYVDGVEVHNAKTKPREEQFNSTYRVVSVLTVLHQDWLNGKEYKCKVSNKGLPSSIEKTISKAKGQPREPQVYTLPPSQEEMTKNQVSLTCLVKGFYPSDIAVEWESNGQPENNYKTTPPVLDSDGSFFLYSRLTVDKSRWQEGNVFSCSVMHEALHNHYTQKSLSLSLGK

SEQ ID NO: 320 - protein, 353 aa, Artificial Sequence
  Synthetic Construct
EVQLVESGGGLVQPGGSLRLSCAASGYIISSYCMGWFRQAPGKGLEGVSAIDSDGGTSYADSVKGRFTISRDNSKNTLYLQMNSLRAEDTAVYYCAADFCWVDEDRHLYEYNSWGQGTLVTVSSESKYGPPCPPCPAPEFLGGPSVFLFPPKPKDTLMISRTPEVTCVVVDVSQEDPEVQFNWYVDGVEVHNAKTKPREEQFNSTYRVVSVLTVLHQDWLNGKEYKCKVSNKGLPSSIEKTISKAKGQPREPQVYTLPPSQEEMTKNQVSLTCLVKGFYPSDIAVEWESNGQPENNYKTTPPVLDSDGSFFLYSRLTVDKSRWQEGNVFSCSVMHEALHNHYTQKSLSLSLGK

SEQ ID NO: 321 - protein, 353 aa, Artificial Sequence
  Synthetic Construct
EVQLVESGGGLVQPGGSLRLSCAASGYIISSYCMGWFRQAPGKGLEGVAAIDSDGGTSYADSVKGRFTISRDNSKNTLYLQMNSLRAEDTAVYYCAADFCWVDEDRHLYEYNSWGQGTLVTVSSESKYGPPCPPCPAPEFLGGPSVFLFPPKPKDTLMISRTPEVTCVVVDVSQEDPEVQFNWYVDGVEVHNAKTKPREEQFNSTYRVVSVLTVLHQDWLNGKEYKCKVSNKGLPSSIEKTISKAKGQPREPQVYTLPPSQEEMTKNQVSLTCLVKGFYPSDIAVEWESNGQPENNYKTTPPVLDSDGSFFLYSRLTVDKSRWQEGNVFSCSVMHEALHNHYTQKSLSLSLGK

SEQ ID NO: 322 - protein, 353 aa, Artificial Sequence
  Synthetic Construct
EVQLVESGGGLVQPGGSLRLSCAASGYIISSYCMGWFRQAPGKGLEGVAAIDSDGGTSYADSVKGRFTISRDNSKNTLYLQMNSLRAEDTAMYYCAADFCWVDEDRHLYEYNSWGQGTLVTVSSESKYGPPCPPCPAPEFLGGPSVFLFPPKPKDTLMISRTPEVTCVVVDVSQEDPEVQFNWYVDGVEVHNAKTKPREEQFNSTYRVVSVLTVLHQDWLNGKEYKCKVSNKGLPSSIEKTISKAKGQPREPQVYTLPPSQEEMTKNQVSLTCLVKGFYPSDIAVEWESNGQPENNYKTTPPVLDSDGSFFLYSRLTVDKSRWQEGNVFSCSVMHEALHNHYTQKSLSLSLGK

SEQ ID NO: 323 - protein, 353 aa, Artificial Sequence
  Synthetic Construct
EVQLVESGGGLVQPGGSLRLSCAASGYIISSYCMGWFRQAPGKGREGVAAIDSDGGTSYADSVKGRFTISRDNSKNTLYLQMNSLRAEDTAMYYCAADFCWVDEDRHLYEYNSWGQGTLVTVSSESKYGPPCPPCPAPEFLGGPSVFLFPPKPKDTLMISRTPEVTCVVVDVSQEDPEVQFNWYVDGVEVHNAKTKPREEQFNSTYRVVSVLTVLHQDWLNGKEYKCKVSNKGLPSSIEKTISKAKGQPREPQVYTLPPSQEEMTKNQVSLTCLVKGFYPSDIAVEWESNGQPENNYKTTPPVLDSDGSFFLYSRLTVDKSRWQEGNVFSCSVMHEALHNHYTQKSLSLSLGK

SEQ ID NO: 324 - protein, 353 aa, Artificial Sequence
  Synthetic Construct
EVQLVESGGGLVQPGGSLRLSCAASGYIISSYCMGWFRQAPGKEREGVAAIDSDGGTSYADSVKGRFTISRDNSKNTLYLQMNSLRAEDTAMYYCAADFCWVDEDRHLYEYNSWGQGTLVTVSSESKYGPPCPPCPAPEFLGGPSVFLFPPKPKDTLMISRTPEVTCVVVDVSQEDPEVQFNWYVDGVEVHNAKTKPREEQFNSTYRVVSVLTVLHQDWLNGKEYKCKVSNKGLPSSIEKTISKAKGQPREPQVYTLPPSQEEMTKNQVSLTCLVKGFYPSDIAVEWESNGQPENNYKTTPPVLDSDGSFFLYSRLTVDKSRWQEGNVFSCSVMHEALHNHYTQKSLSLSLGK

SEQ ID NO: 325 - protein, 353 aa, Artificial Sequence
  Synthetic Construct
EVQLVESGGGLVQPGGSLRLSCAASGYIISSYCMGWFRQAPGKEREGVAAIDSDGGTSYADSVKGRFTISKDNSKNTLYLQMNSLRAEDTAMYYCAADFCWVDEDRHLYEYNSWGQGTLVTVSSESKYGPPCPPCPAPEFLGGPSVFLFPPKPKDTLMISRTPEVTCVVVDVSQEDPEVQFNWYVDGVEVHNAKTKPREEQFNSTYRVVSVLTVLHQDWLNGKEYKCKVSNKGLPSSIEKTISKAKGQPREPQVYTLPPSQEEMTKNQVSLTCLVKGFYPSDIAVEWESNGQPENNYKTTPPVLDSDGSFFLYSRLTVDKSRWQEGNVFSCSVMHEALHNHYTQKSLSLSLGK

SEQ ID NO: 326 - protein, 353 aa, Artificial Sequence
  Synthetic Construct
EVQLVESGGGLVQPGGSLRLSCAASGYIISSYCMGWFRQAPGKGLEGVAAIDSDGGTSYADSVKGRFTISKDNSKNTLYLQMNSLRAEDTAMYYCAADFCWVDEDRHLYEYNSWGQGTLVTVSSESKYGPPCPPCPAPEFLGGPSVFLFPPKPKDTLMISRTPEVTCVVVDVSQEDPEVQFNWYVDGVEVHNAKTKPREEQFNSTYRVVSVLTVLHQDWLNGKEYKCKVSNKGLPSSIEKTISKAKGQPREPQVYTLPPSQEEMTKNQVSLTCLVKGFYPSDIAVEWESNGQPENNYKTTPPVLDSDGSFFLYSRLTVDKSRWQEGNVFSCSVMHEALHNHYTQKSLSLSLGK

SEQ ID NO: 327 - protein, 353 aa, Artificial Sequence
  Synthetic Construct
EVQLVESGGGLVQPGGSLRLSCAASGYIISSYCMGWFRQAPGKGLEGVAAIDSSGGTSYADSVKGRFTISKDNSKNTLYLQMNSLRAEDTAMYYCAADFCWVDEDRHLYEYNSWGQGTLVTVSSESKYGPPCPPCPAPEFLGGPSVFLFPPKPKDTLMISRTPEVTCVVVDVSQEDPEVQFNWYVDGVEVHNAKTKPREEQFNSTYRVVSVLTVLHQDWLNGKEYKCKVSNKGLPSSIEKTISKAKGQPREPQVYTLPPSQEEMTKNQVSLTCLVKGFYPSDIAVEWESNGQPENNYKTTPPVLDSDGSFFLYSRLTVDKSRWQEGNVFSCSVMHEALHNHYTQKSLSLSLGK

SEQ ID NO: 328 - protein, 350 aa, Artificial Sequence
  Synthetic Construct
EVQLVESGGGLVQPGGSLRLSCAASGYTISSYCMGWFRQAPGKGLEGVAAIDSDGSTSYADSVKGRFTISRDNSKNTLYLQMNSLRAEDTAVYYCAADFCWVDDFYEYNYWGQGTLVTVSSESKYGPPCPPCPAPEFLGGPSVFLFPPKPKDTLMISRTPEVTCVVVDVSQEDPEVQFNWYVDGVEVHNAKTKPREEQFNSTYRVVSVLTVLHQDWLNGKEYKCKVSNKGLPSSIEKTISKAKGQPREPQVYTLPPSQEEMTKNQVSLTCLVKGFYPSDIAVEWESNGQPENNYKTTPPVLDSDGSFFLYSRLTVDKSRWQEGNVFSCSVMHEALHNHYTQKSLSLSLGK

SEQ ID NO: 329 - protein, 350 aa, Artificial Sequence
  Synthetic Construct
EVQLVESGGGLVQPGGSLRLSCAASGYTISSYCMGWFRQAPGKGLEGVAAIDSDGSTSYADSVKGRFTISRDNSKNTLYLQMNSLRAEDTAMYYCAADFCWVDDFYEYNYWGQGTLVTVSSESKYGPPCPPCPAPEFLGGPSVFLFPPKPKDTLMISRTPEVTCVVVDVSQEDPEVQFNWYVDGVEVHNAKTKPREEQFNSTYRVVSVLTVLHQDWLNGKEYKCKVSNKGLPSSIEKTISKAKGQPREPQVYTLPPSQEEMTKNQVSLTCLVKGFYPSDIAVEWESNGQPENNYKTTPPVLDSDGSFFLYSRLTVDKSRWQEGNVFSCSVMHEALHNHYTQKSLSLSLGK

SEQ ID NO: 330 - protein, 350 aa, Artificial Sequence
  Synthetic Construct
EVQLVESGGGLVQPGGSLRLSCAASGYTISSYCMGWFRQAPGKGREGVAAIDSDGSTSYADSVKGRFTISRDNSKNTLYLQMNSLRAEDTAMYYCAADFCWVDDFYEYNYWGQGTLVTVSSESKYGPPCPPCPAPEFLGGPSVFLFPPKPKDTLMISRTPEVTCVVVDVSQEDPEVQFNWYVDGVEVHNAKTKPREEQFNSTYRVVSVLTVLHQDWLNGKEYKCKVSNKGLPSSIEKTISKAKGQPREPQVYTLPPSQEEMTKNQVSLTCLVKGFYPSDIAVEWESNGQPENNYKTTPPVLDSDGSFFLYSRLTVDKSRWQEGNVFSCSVMHEALHNHYTQKSLSLSLGK

SEQ ID NO: 331 - protein, 350 aa, Artificial Sequence
  Synthetic Construct
EVQLVESGGGLVQPGGSLRLSCAASGYTISSYCMGWFRQAPGKEREGVAAIDSDGSTSYADSVKGRFTISRDNSKNTLYLQMNSLRAEDTAMYYCAADFCWVDDFYEYNYWGQGTLVTVSSESKYGPPCPPCPAPEFLGGPSVFLFPPKPKDTLMISRTPEVTCVVVDVSQEDPEVQFNWYVDGVEVHNAKTKPREEQFNSTYRVVSVLTVLHQDWLNGKEYKCKVSNKGLPSSIEKTISKAKGQPREPQVYTLPPSQEEMTKNQVSLTCLVKGFYPSDIAVEWESNGQPENNYKTTPPVLDSDGSFFLYSRLTVDKSRWQEGNVFSCSVMHEALHNHYTQKSLSLSLGK

SEQ ID NO: 332 - protein, 350 aa, Artificial Sequence
  Synthetic Construct
EVQLVESGGGLVQPGGSLRLSCAASGYTISSYCMGWFRQAPGKEREGVAAIDSDGSTSYADSVKGRFTISKDNSKNTLYLQMNSLRAEDTAMYYCAADFCWVDDFYEYNYWGQGTLVTVSSESKYGPPCPPCPAPEFLGGPSVFLFPPKPKDTLMISRTPEVTCVVVDVSQEDPEVQFNWYVDGVEVHNAKTKPREEQFNSTYRVVSVLTVLHQDWLNGKEYKCKVSNKGLPSSIEKTISKAKGQPREPQVYTLPPSQEEMTKNQVSLTCLVKGFYPSDIAVEWESNGQPENNYKTTPPVLDSDGSFFLYSRLTVDKSRWQEGNVFSCSVMHEALHNHYTQKSLSLSLGK

SEQ ID NO: 333 - protein, 350 aa, Artificial Sequence
  Synthetic Construct
EVQLVESGGGLVQPGGSLRLSCAASGYTISSYCMGWFRQAPGKGLEGVAAIDSDGSTSYADSVKGRFTISKDNSKNTLYLQMNSLRAEDTAVYYCAADFCWVDDFYEYNYWGQGTLVTVSSESKYGPPCPPCPAPEFLGGPSVFLFPPKPKDTLMISRTPEVTCVVVDVSQEDPEVQFNWYVDGVEVHNAKTKPREEQFNSTYRVVSVLTVLHQDWLNGKEYKCKVSNKGLPSSIEKTISKAKGQPREPQVYTLPPSQEEMTKNQVSLTCLVKGFYPSDIAVEWESNGQPENNYKTTPPVLDSDGSFFLYSRLTVDKSRWQEGNVFSCSVMHEALHNHYTQKSLSLSLGK

SEQ ID NO: 334 - protein, 350 aa, Artificial Sequence
  Synthetic Construct
EVQLVESGGGLVQPGGSLRLSCAASGYTISSYCMGWFRQAPGKGLEGVAAIDSSGSTSYADSVKGRFTISKDNSKNTLYLQMNSLRAEDTAVYYCAADFCWVDDFYEYNYWGQGTLVTVSSESKYGPPCPPCPAPEFLGGPSVFLFPPKPKDTLMISRTPEVTCVVVDVSQEDPEVQFNWYVDGVEVHNAKTKPREEQFNSTYRVVSVLTVLHQDWLNGKEYKCKVSNKGLPSSIEKTISKAKGQPREPQVYTLPPSQEEMTKNQVSLTCLVKGFYPSDIAVEWESNGQPENNYKTTPPVLDSDGSFFLYSRLTVDKSRWQEGNVFSCSVMHEALHNHYTQKSLSLSLGK

SEQ ID NO: 335 - protein, 351 aa, Artificial Sequence
  Synthetic Construct
EVQLVESGGGLVQPGGSLRLSCAASGYTVSSYCMGWFRQAPGKGLEGVSAIDSDGSVSYADSVKGRFTISRDNSKNTLYLQMNSLRAEDTAVYYCAADLCWVDQDQGEYNTWGQGTLVTVSSESKYGPPCPPCPAPEFLGGPSVFLFPPKPKDTLMISRTPEVTCVVVDVSQEDPEVQFNWYVDGVEVHNAKTKPREEQFNSTYRVVSVLTVLHQDWLNGKEYKCKVSNKGLPSSIEKTISKAKGQPREPQVYTLPPSQEEMTKNQVSLTCLVKGFYPSDIAVEWESNGQPENNYKTTPPVLDSDGSFFLYSRLTVDKSRWQEGNVFSCSVMHEALHNHYTQKSLSLSLGK

SEQ ID NO: 336 - protein, 351 aa, Artificial Sequence
  Synthetic Construct
EVQLVESGGGLVQPGGSLRLSCAASGYTVSSYCMGWFRQAPGKGLEGVSAIDSDGSVSYADSVKGRFTISRDNSKNTLYLQMNSLRAEDTAVYFCAADLCWVDQDQGEYNTWGQGTLVTVSSESKYGPPCPPCPAPEFLGGPSVFLFPPKPKDTLMISRTPEVTCVVVDVSQEDPEVQFNWYVDGVEVHNAKTKPREEQFNSTYRVVSVLTVLHQDWLNGKEYKCKVSNKGLPSSIEKTISKAKGQPREPQVYTLPPSQEEMTKNQVSLTCLVKGFYPSDIAVEWESNGQPENNYKTTPPVLDSDGSFFLYSRLTVDKSRWQEGNVFSCSVMHEALHNHYTQKSLSLSLGK

SEQ ID NO: 337 - protein, 351 aa, Artificial Sequence
  Synthetic Construct
EVQLVESGGGLVQPGGSLRLSCAASGYTVSSYCMGWFRQAPGKGLEGVAAIDSDGSVSYADSVKGRFTISRDNSKNTLYLQMNSLRAEDTAVYFCAADLCWVDQDQGEYNTWGQGTLVTVSSESKYGPPCPPCPAPEFLGGPSVFLFPPKPKDTLMISRTPEVTCVVVDVSQEDPEVQFNWYVDGVEVHNAKTKPREEQFNSTYRVVSVLTVLHQDWLNGKEYKCKVSNKGLPSSIEKTISKAKGQPREPQVYTLPPSQEEMTKNQVSLTCLVKGFYPSDIAVEWESNGQPENNYKTTPPVLDSDGSFFLYSRLTVDKSRWQEGNVFSCSVMHEALHNHYTQKSLSLSLGK

SEQ ID NO: 338 - protein, 351 aa, Artificial Sequence
  Synthetic Construct
EVQLVESGGGLVQPGGSLRLSCAASGYTVSSYCMGWFRQAPGKGLEGVAAIDSDGSVSYADSVKGRFTISRDNSKNTLYLQMNSLRAEDTAMYFCAADLCWVDQDQGEYNTWGQGTLVTVSSESKYGPPCPPCPAPEFLGGPSVFLFPPKPKDTLMISRTPEVTCVVVDVSQEDPEVQFNWYVDGVEVHNAKTKPREEQFNSTYRVVSVLTVLHQDWLNGKEYKCKVSNKGLPSSIEKTISKAKGQPREPQVYTLPPSQEEMTKNQVSLTCLVKGFYPSDIAVEWESNGQPENNYKTTPPVLDSDGSFFLYSRLTVDKSRWQEGNVFSCSVMHEALHNHYTQKSLSLSLGK

SEQ ID NO: 339 - protein, 351 aa, Artificial Sequence
  Synthetic Construct
EVQLVESGGGLVQPGGSLRLSCAASGYTVSSYCMGWFRQAPGKGREGVAAIDSDGSVSYADSVKGRFTISRDNSKNTLYLQMNSLRAEDTAMYFCAADLCWVDQDQGEYNTWGQGTLVTVSSESKYGPPCPPCPAPEFLGGPSVFLFPPKPKDTLMISRTPEVTCVVVDVSQEDPEVQFNWYVDGVEVHNAKTKPREEQFNSTYRVVSVLTVLHQDWLNGKEYKCKVSNKGLPSSIEKTISKAKGQPREPQVYTLPPSQEEMTKNQVSLTCLVKGFYPSDIAVEWESNGQPENNYKTTPPVLDSDGSFFLYSRLTVDKSRWQEGNVFSCSVMHEALHNHYTQKSLSLSLGK

SEQ ID NO: 340 - protein, 351 aa, Artificial Sequence
  Synthetic Construct
EVQLVESGGGLVQPGGSLRLSCAASGYTVSSYCMGWFRQAPGKEREGVAAIDSDGSVSYADSVKGRFTISRDNSKNTLYLQMNSLRAEDTAMYFCAADLCWVDQDQGEYNTWGQGTLVTVSSESKYGPPCPPCPAPEFLGGPSVFLFPPKPKDTLMISRTPEVTCVVVDVSQEDPEVQFNWYVDGVEVHNAKTKPREEQFNSTYRVVSVLTVLHQDWLNGKEYKCKVSNKGLPSSIEKTISKAKGQPREPQVYTLPPSQEEMTKNQVSLTCLVKGFYPSDIAVEWESNGQPENNYKTTPPVLDSDGSFFLYSRLTVDKSRWQEGNVFSCSVMHEALHNHYTQKSLSLSLGK

SEQ ID NO: 341 - protein, 351 aa, Artificial Sequence
  Synthetic Construct
EVQLVESGGGLVQPGGSLRLSCAASGYTVSSYCMGWFRQAPGKEREGVAAIDSDGSVSYADSVKGRFTISKDNSKNTLYLQMNSLRAEDTAMYFCAADLCWVDQDQGEYNTWGQGTLVTVSSESKYGPPCPPCPAPEFLGGPSVFLFPPKPKDTLMISRTPEVTCVVVDVSQEDPEVQFNWYVDGVEVHNAKTKPREEQFNSTYRVVSVLTVLHQDWLNGKEYKCKVSNKGLPSSIEKTISKAKGQPREPQVYTLPPSQEEMTKNQVSLTCLVKGFYPSDIAVEWESNGQPENNYKTTPPVLDSDGSFFLYSRLTVDKSRWQEGNVFSCSVMHEALHNHYTQKSLSLSLGK

SEQ ID NO: 342 - protein, 351 aa, Artificial Sequence
  Synthetic Construct
EVQLVESGGGLVQPGGSLRLSCAASGYTVSSYCMGWFRQAPGKGREGVSAIDSDGSVSYADSVKGRFTISKDNSKNTLYLQMNSLRAEDTAVYFCAADLCWVDQDQGEYNTWGQGTLVTVSSESKYGPPCPPCPAPEFLGGPSVFLFPPKPKDTLMISRTPEVTCVVVDVSQEDPEVQFNWYVDGVEVHNAKTKPREEQFNSTYRVVSVLTVLHQDWLNGKEYKCKVSNKGLPSSIEKTISKAKGQPREPQVYTLPPSQEEMTKNQVSLTCLVKGFYPSDIAVEWESNGQPENNYKTTPPVLDSDGSFFLYSRLTVDKSRWQEGNVFSCSVMHEALHNHYTQKSLSLSLGK

SEQ ID NO: 343 - protein, 351 aa, Artificial Sequence
  Synthetic Construct
EVQLVESGGGLVQPGGSLRLSCAASGYTVSSYCMGWFRQAPGKGREGVSAIDSSGSVSYADSVKGRFTISKDNSKNTLYLQMNSLRAEDTAVYFCAADLCWVDQDQGEYNTWGQGTLVTVSSESKYGPPCPPCPAPEFLGGPSVFLFPPKPKDTLMISRTPEVTCVVVDVSQEDPEVQFNWYVDGVEVHNAKTKPREEQFNSTYRVVSVLTVLHQDWLNGKEYKCKVSNKGLPSSIEKTISKAKGQPREPQVYTLPPSQEEMTKNQVSLTCLVKGFYPSDIAVEWESNGQPENNYKTTPPVLDSDGSFFLYSRLTVDKSRWQEGNVFSCSVMHEALHNHYTQKSLSLSLGK

SEQ ID NO: 344 - protein, 355 aa, Artificial Sequence
  Synthetic Construct
EVQLVESGGGLVQPGGSLRLSCAASGYTYGGYCMGWFRQAPGKGLEGVSTINSDGSTNYADSVKGRFTISRDNSKNTLYLQMNSLRAEDTAVYYCAVDLAPCWVAGPIEAADFGYWGQGTLVTVSSESKYGPPCPPCPAPEFLGGPSVFLFPPKPKDTLMISRTPEVTCVVVDVSQEDPEVQFNWYVDGVEVHNAKTKPREEQFNSTYRVVSVLTVLHQDWLNGKEYKCKVSNKGLPSSIEKTISKAKGQPREPQVYTLPPSQEEMTKNQVSLTCLVKGFYPSDIAVEWESNGQPENNYKTTPPVLDSDGSFFLYSRLTVDKSRWQEGNVFSCSVMHEALHNHYTQKSLSLSLGK

SEQ ID NO: 345 - protein, 355 aa, Artificial Sequence
  Synthetic Construct
EVQLVESGGGLVQPGGSLRLSCAASGYTYGGYCMGWFRQAPGKGLEGVSTIASEGSTNYADSVKGRFTISRDNSKNTLYLQMNSLRAEDTAVYYCAVDLAPCWVAGPIEAADFGYWGQGTLVTVSSESKYGPPCPPCPAPEFLGGPSVFLFPPKPKDTLMISRTPEVTCVVVDVSQEDPEVQFNWYVDGVEVHNAKTKPREEQFNSTYRVVSVLTVLHQDWLNGKEYKCKVSNKGLPSSIEKTISKAKGQPREPQVYTLPPSQEEMTKNQVSLTCLVKGFYPSDIAVEWESNGQPENNYKTTPPVLDSDGSFFLYSRLTVDKSRWQEGNVFSCSVMHEALHNHYTQKSLSLSLGK

SEQ ID NO: 346 - protein, 355 aa, Artificial Sequence
  Synthetic Construct
EVQLVESGGGLVQPGGSLRLSCAASGYTYGGYCMGWFRQAPGKGLEGVSTIASSGSTNYADSVKGRFTISRDNSKNTLYLQMNSLRAEDTAVYYCAVDLAPCWVAGPIEAADFGYWGQGTLVTVSSESKYGPPCPPCPAPEFLGGPSVFLFPPKPKDTLMISRTPEVTCVVVDVSQEDPEVQFNWYVDGVEVHNAKTKPREEQFNSTYRVVSVLTVLHQDWLNGKEYKCKVSNKGLPSSIEKTISKAKGQPREPQVYTLPPSQEEMTKNQVSLTCLVKGFYPSDIAVEWESNGQPENNYKTTPPVLDSDGSFFLYSRLTVDKSRWQEGNVFSCSVMHEALHNHYTQKSLSLSLGK

SEQ ID NO: 347 - protein, 355 aa, Artificial Sequence
  Synthetic Construct
EVQLVESGGGLVQPGGSLRLSCAASGYTYGGYCMGWFRQAPGKGREGVSTINSDGSTNYADSVKGRFTISRDNAKNTLYLQMNSLRPEDTAVYYCAVDLAPCWVAGPIEAADFGYWGQGTLVTVSSESKYGPPCPPCPAPEFLGGPSVFLFPPKPKDTLMISRTPEVTCVVVDVSQEDPEVQFNWYVDGVEVHNAKTKPREEQFNSTYRVVSVLTVLHQDWLNGKEYKCKVSNKGLPSSIEKTISKAKGQPREPQVYTLPPSQEEMTKNQVSLTCLVKGFYPSDIAVEWESNGQPENNYKTTPPVLDSDGSFFLYSRLTVDKSRWQEGNVFSCSVMHEALHNHYTQKSLSLSLGK

SEQ ID NO: 348 - protein, 355 aa, Artificial Sequence
  Synthetic Construct
EVQLVESGGGLVQPGGSLRLSCAASGYTYGGYCMGWFRQAPGKGREGVSTIASEGSTNYADSVKGRFTISRDNAKNTLYLQMNSLRPEDTAVYYCAVDLAPCWVAGPIEAADFGYWGQGTLVTVSSESKYGPPCPPCPAPEFLGGPSVFLFPPKPKDTLMISRTPEVTCVVVDVSQEDPEVQFNWYVDGVEVHNAKTKPREEQFNSTYRVVSVLTVLHQDWLNGKEYKCKVSNKGLPSSIEKTISKAKGQPREPQVYTLPPSQEEMTKNQVSLTCLVKGFYPSDIAVEWESNGQPENNYKTTPPVLDSDGSFFLYSRLTVDKSRWQEGNVFSCSVMHEALHNHYTQKSLSLSLGK

SEQ ID NO: 349 - protein, 355 aa, Artificial Sequence
  Synthetic Construct
EVQLVESGGGLVQPGGSLRLSCAASGYTYGGYCMGWFRQAPGKGREGVSTIASSGSTNYADSVKGRFTISRDNAKNTLYLQMNSLRPEDTAVYYCAVDLAPCWVAGPIEAADFGYWGQGTLVTVSSESKYGPPCPPCPAPEFLGGPSVFLFPPKPKDTLMISRTPEVTCVVVDVSQEDPEVQFNWYVDGVEVHNAKTKPREEQFNSTYRVVSVLTVLHQDWLNGKEYKCKVSNKGLPSSIEKTISKAKGQPREPQVYTLPPSQEEMTKNQVSLTCLVKGFYPSDIAVEWESNGQPENNYKTTPPVLDSDGSFFLYSRLTVDKSRWQEGNVFSCSVMHEALHNHYTQKSLSLSLGK

SEQ ID NO: 350 - protein, 497 aa, Artificial Sequence
  Synthetic Construct
VPVVWAQEGAPAQLPCSPTIPLQDLSLLRRAGVTWQHQPDSGPPAAAPGHPLAPGPHPAAPSSWGPRPRRYTVLSVGPGGLRSGRLPLQPRVQLDERGRQRGDFSLWLRPARRADAGEYRAAVHLRDRALSCRLRLRLGQASMTASPPGSLRASDWVILNCSFSRPDRPASVHWFRNRGQGRVPVRESPHHHLAESFLFLPQVSPMDSGPWGCILTYRDGFNVSIMYNLTVLGLEPPTPLTVYAGAGSRVGLPCRLPAGVGTRSFLTAKWTPPGGGPDLLVTGDNGDFTLRLEDVSQAQAGTYTCHIHLQEQQLNATVTLAIITVTPKSFGSPGSLGKLLCEVTPVSGQERFVWSSLDTPSQRSFSGPWLEAQEAQLLSQPWQCQLYQGERLLGAAVYFTELSSPGAQRSGRAPGALPAGHLLLFLILGVLSLLLLVTGAFGFHLWRRQWRPRRFSALEQGIHPPQAQSKIEELEQEPEPEPEPEPEPEPEPEPEQL

SEQ ID NO: 351 - protein, 422 aa, Artificial Sequence
  Synthetic Construct
VPVVWAQEGAPAQLPCSPTIPLQDLSLLRRAGVTWQHQPDSGPPAAAPGHPLAPGPHPAAPSSWGPRPRRYTVLSVGPGGLRSGRLPLQPRVQLDERGRQRGDFSLWLRPARRADAGEYRAAVHLRDRALSCRLRLRLGQASMTASPPGSLRASDWVILNCSFSRPDRPASVHWFRNRGQGRVPVRESPHHHLAESFLFLPQVSPMDSGPWGCILTYRDGFNVSIMYNLTVLGLEPPTPLTVYAGAGSRVGLPCRLPAGVGTRSFLTAKWTPPGGGPDLLVTGDNGDFTLRLEDVSQAQAGTYTCHIHLQEQQLNATVTLAIITVTPKSFGSPGSLGKLLCEVTPVSGQERFVWSSLDTPSQRSFSGPWLEAQEAQLLSQPWQCQLYQGERLLGAAVYFTELSSPGAQRSGRAPGALPAGHL

SEQ ID NO: 352 - protein, 15 aa, Artificial Sequence
  Synthetic Construct
EPKSSDKTHTCPPCP

SEQ ID NO: 353 - protein, 15 aa, Artificial Sequence
  Synthetic Construct
EPKSSDKTHTSPPSP

SEQ ID NO: 354 - protein, 447 aa, Artificial Sequence
  Synthetic Construct
QVQLQQWGAGLLKPSETLSLTCAVYGGSFSDYYWNWIRQPPGKGLEWIGEINHRGSTNSNPSLKSRVTLSLDTSKNQFSLKLRSVTAADTAVYYCAFGYSDYEYNWFDPWGQGTLVTVSSASTKGPSVFPLAPCSRSTSESTAALGCLVKDYFPEPVTVSWNSGALTSGVHTFPAVLQSSGLYSLSSVVTVPSSSLGTKTYTCNVDHKPSNTKVDKRVESKYGPPCPPCPAPEFLGGPSVFLFPPKPKDTLMISRTPEVTCVVVDVSQEDPEVQFNWYVDGVEVHNAKTKPREEQFNSTYRVVSVLTVLHQDWLNGKEYKCKVSNKGLPSSIEKTISKAKGQPREPQVYTLPPSQEEMTKNQVSLTCLVKGFYPSDIAVEWESNGQPENNYKTTPPVLDSDGSFFLYSRLTVDKSRWQEGNVFSCSVMHEALHNHYTQKSLSLSLGK

SEQ ID NO: 355 - protein, 214 aa, Artificial Sequence
  Synthetic Construct
EIVLTQSPATLSLSPGERATLSCRASQSISSYLAWYQQKPGQAPRLLIYDASNRATGIPARFSGSGSGTDFTLTISSLEPEDFAVYYCQQRSNWPLTFGQGTNLEIKRTVAAPSVFIFPPSDEQLKSGTASVVCLLNNFYPREAKVQWKVDNALQSGNSQESVTEQDSKDSTYSLSSTLTLSKADYEKHKVYACEVTHQGLSSPVTKSFNRGEC

SEQ ID NO: 356 - protein, 447 aa, Artificial Sequence
  Synthetic Construct
QVQLVQSGVEVKKPGASVKVSCKASGYTFTNYYMYWVRQAPGQGLEWMGGINPSNGGTNFNEKFKNRVTLTTDSSTTTAYMELKSLQFDDTAVYYCARRDYRFDMGFDYWGQGTTVTVSSASTKGPSVFPLAPCSRSTSESTAALGCLVKDYFPEPVTVSWNSGALTSGVHTFPAVLQSSGLYSLSSVVTVPSSSLGTKTYTCNVDHKPSNTKVDKRVESKYGPPCPPCPAPEFLGGPSVFLFPPKPKDTLMISRTPEVTCVVVDVSQEDPEVQFNWYVDGVEVHNAKTKPREEQFNSTYRVVSVLTVLHQDWLNGKEYKCKVSNKGLPSSIEKTISKAKGQPREPQVYTLPPSQEEMTKNQVSLTCLVKGFYPSDIAVEWESNGQPENNYKTTPPVLDSDGSFFLYSRLTVDKSRWQEGNVFSCSVMHEALHNHYTQKSLSLSLGK

SEQ ID NO: 357 - protein, 218 aa, Artificial Sequence
  Synthetic Construct
EIVLTQSPATLSLSPGERATLSCRASKGVSTSGYSYLHWYQQKPGQAPRLLIYLASYLESGVPARFSGSGSGTDFTLTISSLEPEDFAVYYCQHSRDLPLTFGGGTKVEIKRTVAAPSVFIFPPSDEQLKSGTASVVCLLNNFYPREAKVQWKVDNALQSGNSQESVTEQDSKDSTYSLSSTLTLSKADYEKHKVYACEVTHQGLSSPVTKSFNRGEC

SEQ ID NO: 358 - protein, 584 aa, Artificial Sequence
  Synthetic Construct
EVQLVESGGGLVQPGGSLRLSCAASGYTVSSYCMGWFRQAPGKGREGVSAIDSDGSVSYADSVKGRFTISKDNSKNTLYLQMNSLRAEDTAVYFCAADLCWVDQDQGEYNTWGQGTLVTVSSEPKSSDKTHTSPPSPQVQLVQSGVEVKKPGASVKVSCKASGYTFTNYYMYWVRQAPGQGLEWMGGINPSNGGTNFNEKFKNRVTLTTDSSTTTAYMELKSLQFDDTAVYYCARRDYRFDMGFDYWGQGTTVTVSSASTKGPSVFPLAPCSRSTSESTAALGCLVKDYFPEPVTVSWNSGALTSGVHTFPAVLQSSGLYSLSSVVTVPSSSLGTKTYTCNVDHKPSNTKVDKRVESKYGPPCPPCPAPEFLGGPSVFLFPPKPKDTLMISRTPEVTCVVVDVSQEDPEVQFNWYVDGVEVHNAKTKPREEQFNSTYRVVSVLTVLHQDWLNGKEYKCKVSNKGLPSSIEKTISKAKGQPREPQVYTLPPSQEEMTKNQVSLTCLVKGFYPSDIAVEWESNGQPENNYKTTPPVLDSDGSFFLYSRLTVDKSRWQEGNVFSCSVMHEALHNHYTQKSLSLSLGK

SEQ ID NO: 359 - protein, 218 aa, Artificial Sequence; identical to SEQ ID NO: 357
  Synthetic Construct

SEQ ID NO: 360 - protein, 447 aa, Artificial Sequence; identical to SEQ ID NO: 356
  Synthetic Construct

SEQ ID NO: 361 - protein, 355 aa, Artificial Sequence
  Synthetic Construct
EVQLVESGGGLVQPGGSLRLSCAASGYTVSSYCMGWFRQAPGKGREGVSAIDSDGSVSYADSVKGRFTISKDNSKNTLYLQMNSLRAEDTAVYFCAADLCWVDQDQGEYNTWGQGTLVTVSSEPKSSDKTHTSPPSPEIVLTQSPATLSLSPGERATLSCRASKGVSTSGYSYLHWYQQKPGQAPRLLIYLASYLESGVPARFSGSGSGTDFTLTISSLEPEDFAVYYCQHSRDLPLTFGGGTKVEIKRTVAAPSVFIFPPSDEQLKSGTASVVCLLNNFYPREAKVQWKVDNALQSGNSQESVTEQDSKDSTYSLSSTLTLSKADYEKHKVYACEVTHQGLSSPVTKSFNRGEC

SEQ ID NO: 362 - protein, 588 aa, Artificial Sequence
  Synthetic Construct
EVQLVESGGGLVQPGGSLRLSCAASGYTYGGYCMGWFRQAPGKGLEGVSTINSDGSTNYADSVKGRFTISRDNSKNTLYLQMNSLRAEDTAVYYCAVDLAPCWVAGPIEAADFGYWGQGTLVTVSSEPKSSDKTHTSPPSPQVQLVQSGVEVKKPGASVKVSCKASGYTFTNYYMYWVRQAPGQGLEWMGGINPSNGGTNFNEKFKNRVTLTTDSSTTTAYMELKSLQFDDTAVYYCARRDYRFDMGFDYWGQGTTVTVSSASTKGPSVFPLAPCSRSTSESTAALGCLVKDYFPEPVTVSWNSGALTSGVHTFPAVLQSSGLYSLSSVVTVPSSSLGTKTYTCNVDHKPSNTKVDKRVESKYGPPCPPCPAPEFLGGPSVFLFPPKPKDTLMISRTPEVTCVVVDVSQEDPEVQFNWYVDGVEVHNAKTKPREEQFNSTYRVVSVLTVLHQDWLNGKEYKCKVSNKGLPSSIEKTISKAKGQPREPQVYTLPPSQEEMTKNQVSLTCLVKGFYPSDIAVEWESNGQPENNYKTTPPVLDSDGSFFLYSRLTVDKSRWQEGNVFSCSVMHEALHNHYTQKSLSLSLGK

SEQ ID NO: 363 - protein, 218 aa, Artificial Sequence; identical to SEQ ID NO: 357
  Synthetic Construct

SEQ ID NO: 364 - protein, 447 aa, Artificial Sequence; identical to SEQ ID NO: 356
  Synthetic Construct

SEQ ID NO: 365 - protein, 359 aa, Artificial Sequence
  Synthetic Construct
EVQLVESGGGLVQPGGSLRLSCAASGYTYGGYCMGWFRQAPGKGLEGVSTINSDGSTNYADSVKGRFTISRDNSKNTLYLQMNSLRAEDTAVYYCAVDLAPCWVAGPIEAADFGYWGQGTLVTVSSEPKSSDKTHTSPPSPEIVLTQSPATLSLSPGERATLSCRASKGVSTSGYSYLHWYQQKPGQAPRLLIYLASYLESGVPARFSGSGSGTDFTLTISSLEPEDFAVYYCQHSRDLPLTFGGGTKVEIKRTVAAPSVFIFPPSDEQLKSGTASVVCLLNNFYPREAKVQWKVDNALQSGNSQESVTEQDSKDSTYSLSSTLTLSKADYEKHKVYACEVTHQGLSSPVTKSFNRGEC

SEQ ID NO: 366 - protein, 9 aa, Artificial Sequence
  Synthetic Construct
GGGGSGGGS

SEQ ID NO: 367 - protein, 15 aa, Artificial Sequence
  Synthetic Construct
GGGGSGGGGSGGGGS

SEQ ID NO: 368 - protein, 1 aa, Artificial Sequence
  Synthetic Construct
  VARIANT 1: can be present in repeat of at least 1
G

SEQ ID NO: 369 - protein, 2 aa, Artificial Sequence
  Synthetic Construct
  VARIANT (1)..(2): can be present in repeat of at least 1
GS

SEQ ID NO: 370 - protein, 5 aa, Artificial Sequence
  Synthetic Construct
  VARIANT (1)..(5): can be present in repeat of at least 1
GSGGS

SEQ ID NO: 371 - protein, 4 aa, Artificial Sequence
  Synthetic Construct
  VARIANT (1)..(4): can be present in repeat of at least 1
GGGS

SEQ ID NO: 372 - protein, 5 aa, Artificial Sequence
  Synthetic Construct
  VARIANT (1)..(5): can be present in repeat of at least 1
GGGGS

SEQ ID NO: 373 - protein, 444 aa, Artificial Sequence
  Synthetic Construct
EVQLVESGGGLVQPGGSLRLSCAASGFVFSRYDMAWVRQAPGKGLEWVSFISGGGSNTYYPDTVKGRFTISRDNSKNTLYLQMNSLRAEDTAVYYCISPYYYAMEYWGQGTTVTVSSASTKGPSVFPLAPCSRSTSESTAALGCLVKDYFPEPVTVSWNSGALTSGVHTFPAVLQSSGLYSLSSVVTVPSSSLGTKTYTCNVDHKPSNTKVDKRVESKYGPPCPPCPAPEFLGGPSVFLFPPKPKDTLMISRTPEVTCVVVDVSQEDPEVQFNWYVDGVEVHNAKTKPREEQFNSTYRVVSVLTVLHQDWLNGKEYKCKVSNKGLPSSIEKTISKAKGQPREPQVYTLPPSQEEMTKNQVSLTCLVKGFYPSDIAVEWESNGQPENNYKTTPPVLDSDGSFFLYSRLTVDKSRWQEGNVFSCSVMHEALHNHYTQKSLSLSLGK

SEQ ID NO: 374 - protein, 214 aa, Artificial Sequence
  Synthetic Construct
DIQMTQSPSSVSASVGDRVTITCKASQDVDTAVAWYQQKPGKAPKLLIYWASTRHTGVPSRFSGSGSGTDFTLTISSLQPEDFATYYCQQYSTFPWTFGGGTKVEIKRTVAAPSVFIFPPSDEQLKSGTASVVCLLNNFYPREAKVQWKVDNALQSGNSQESVTEQDSKDSTYSLSSTLTLSKADYEKHKVYACEVTHQGLSSPVTKSFNRGEC

SEQ ID NO: 375 - protein, 583 aa, Artificial Sequence
  Synthetic Construct
EVQLVESGGGSVQAGGSLRLSCAASGYIISSYCMGWFRQAPGKEREGVAAIDSDGGTSYADSVKGRFTISKDNAKNTLYLQMDSLKPEDTAMYYCAADFCWVDEDRHLYEYNSWGQGTQVTVSSEPKSSDKTHTSPPSPEVQLVESGGGLVQPGGSLRLSCAASGFVFSRYDMAWVRQAPGKGLEWVSFISGGGSNTYYPDTVKGRFTISRDNSKNTLYLQMNSLRAEDTAVYYCISPYYYAMEYWGQGTTVTVSSASTKGPSVFPLAPCSRSTSESTAALGCLVKDYFPEPVTVSWNSGALTSGVHTFPAVLQSSGLYSLSSVVTVPSSSLGTKTYTCNVDHKPSNTKVDKRVESKYGPPCPPCPAPEFLGGPSVFLFPPKPKDTLMISRTPEVTCVVVDVSQEDPEVQFNWYVDGVEVHNAKTKPREEQFNSTYRVVSVLTVLHQDWLNGKEYKCKVSNKGLPSSIEKTISKAKGQPREPQVYTLPPSQEEMTKNQVSLTCLVKGFYPSDIAVEWESNGQPENNYKTTPPVLDSDGSFFLYSRLTVDKSRWQEGNVFSCSVMHEALHNHYTQKSLSLSLGK

SEQ ID NO: 376 - protein, 214 aa, Artificial Sequence; identical to SEQ ID NO: 374
  Synthetic Construct

SEQ ID NO: 377 - protein, 580 aa, Artificial Sequence
  Synthetic Construct
QVQLAESGGGSVQAGGSLRLSCAASGYTISSYCMGWFRQAPGKEREGVAAIDSDGSTSYADSVKGRFTISKDNAKNTLYLQMNSLKPEDTAMYYCAADFCWVDDFYEYNYWGQGTQVTVSSEPKSSDKTHTSPPSPEVQLVESGGGLVQPGGSLRLSCAASGFVFSRYDMAWVRQAPGKGLEWVSFISGGGSNTYYPDTVKGRFTISRDNSKNTLYLQMNSLRAEDTAVYYCISPYYYAMEYWGQGTTVTVSSASTKGPSVFPLAPCSRSTSESTAALGCLVKDYFPEPVTVSWNSGALTSGVHTFPAVLQSSGLYSLSSVVTVPSSSLGTKTYTCNVDHKPSNTKVDKRVESKYGPPCPPCPAPEFLGGPSVFLFPPKPKDTLMISRTPEVTCVVVDVSQEDPEVQFNWYVDGVEVHNAKTKPREEQFNSTYRVVSVLTVLHQDWLNGKEYKCKVSNKGLPSSIEKTISKAKGQPREPQVYTLPPSQEEMTKNQVSLTCLVKGFYPSDIAVEWESNGQPENNYKTTPPVLDSDGSFFLYSRLTVDKSRWQEGNVFSCSVMHEALHNHYTQKSLSLSLGK

SEQ ID NO: 378 - protein, 214 aa, Artificial Sequence; identical to SEQ ID NO: 374
  Synthetic Construct

SEQ ID NO: 379 - protein, 585 aa, Artificial Sequence
  Synthetic Construct
EVQLAESGGGSVQAGGSLRLSCAASGYTYGGYCMGWFRQAPGKEREGVATINSDGSTNYADSVKGRFTISKDNAKNTLYLQMNSLSPEDTAMYYCAVDLAPCWVAGPIEAADFGYWGQGTQVTVSSEPKSSDKTHTSPPSPEVQLVESGGGLVQPGGSLRLSCAASGFVFSRYDMAWVRQAPGKGLEWVSFISGGGSNTYYPDTVKGRFTISRDNSKNTLYLQMNSLRAEDTAVYYCISPYYYAMEYWGQGTTVTVSSASTKGPSVFPLAPCSRSTSESTAALGCLVKDYFPEPVTVSWNSGALTSGVHTFPAVLQSSGLYSLSSVVTVPSSSLGTKTYTCNVDHKPSNTKVDKRVESKYGPPCPPCPAPEFLGGPSVFLFPPKPKDTLMISRTPEVTCVVVDVSQEDPEVQFNWYVDGVEVHNAKTKPREEQFNSTYRVVSVLTVLHQDWLNGKEYKCKVSNKGLPSSIEKTISKAKGQPREPQVYTLPPSQEEMTKNQVSLTCLVKGFYPSDIAVEWESNGQPENNYKTTPPVLDSDGSFFLYSRLTVDKSRWQEGNVFSCSVMHEALHNHYTQKSLSLSLGK

SEQ ID NO: 380 - protein, 214 aa, Artificial Sequence; identical to SEQ ID NO: 374
  Synthetic Construct

SEQ ID NO: 381 - protein, 581 aa, Artificial Sequence
  Synthetic Construct
QVHLMESGGGSVQVGGSLRLSCAASGYTVSSYCMGWFRQAPGKEREGVAAIDSDGSVSYADSVKGRFTISKDNAKNTLYLQMNSLKPEDTAMYFCAADLCWVDQDQGEYNTWGQGTQVTVSSEPKSSDKTHTSPPSPEVQLVESGGGLVQPGGSLRLSCAASGFVFSRYDMAWVRQAPGKGLEWVSFISGGGSNTYYPDTVKGRFTISRDNSKNTLYLQMNSLRAEDTAVYYCISPYYYAMEYWGQGTTVTVSSASTKGPSVFPLAPCSRSTSESTAALGCLVKDYFPEPVTVSWNSGALTSGVHTFPAVLQSSGLYSLSSVVTVPSSSLGTKTYTCNVDHKPSNTKVDKRVESKYGPPCPPCPAPEFLGGPSVFLFPPKPKDTLMISRTPEVTCVVVDVSQEDPEVQFNWYVDGVEVHNAKTKPREEQFNSTYRVVSVLTVLHQDWLNGKEYKCKVSNKGLPSSIEKTISKAKGQPREPQVYTLPPSQEEMTKNQVSLTCLVKGFYPSDIAVEWESNGQPENNYKTTPPVLDSDGSFFLYSRLTVDKSRWQEGNVFSCSVMHEALHNHYTQKSLSLSLGK

SEQ ID NO: 382 - protein, 214 aa, Artificial Sequence; identical to SEQ ID NO: 374
  Synthetic Construct

SEQ ID NO: 383 - protein, 583 aa, Artificial Sequence
  Synthetic Construct
EVQLVESGGGLVQPGGSLRLSCAASGYIISSYCMGWFRQAPGKGLEGVAAIDSDGGTSYADSVKGRFTISKDNSKNTLYLQMNSLRAEDTAMYYCAADFCWVDEDRHLYEYNSWGQGTLVTVSSEPKSSDKTHTSPPSPEVQLVESGGGLVQPGGSLRLSCAASGFVFSRYDMAWVRQAPGKGLEWVSFISGGGSNTYYPDTVKGRFTISRDNSKNTLYLQMNSLRAEDTAVYYCISPYYYAMEYWGQGTTVTVSSASTKGPSVFPLAPCSRSTSESTAALGCLVKDYFPEPVTVSWNSGALTSGVHTFPAVLQSSGLYSLSSVVTVPSSSLGTKTYTCNVDHKPSNTKVDKRVESKYGPPCPPCPAPEFLGGPSVFLFPPKPKDTLMISRTPEVTCVVVDVSQEDPEVQFNWYVDGVEVHNAKTKPREEQFNSTYRVVSVLTVLHQDWLNGKEYKCKVSNKGLPSSIEKTISKAKGQPREPQVYTLPPSQEEMTKNQVSLTCLVKGFYPSDIAVEWESNGQPENNYKTTPPVLDSDGSFFLYSRLTVDKSRWQEGNVFSCSVMHEALHNHYTQKSLSLSLGK

SEQ ID NO: 384 - protein, 214 aa, Artificial Sequence; identical to SEQ ID NO: 374
  Synthetic Construct

SEQ ID NO: 385 - protein, 583 aa, Artificial Sequence
  Synthetic Construct
EVQLVESGGGLVQPGGSLRLSCAASGFVFSRYDMAWVRQAPGKGLEWVSFISGGGSNTYYPDTVKGRFTISRDNSKNTLYLQMNSLRAEDTAVYYCISPYYYAMEYWGQGTTVTVSSASTKGPSVFPLAPCSRSTSESTAALGCLVKDYFPEPVTVSWNSGALTSGVHTFPAVLQSSGLYSLSSVVTVPSSSLGTKTYTCNVDHKPSNTKVDKRVESKYGPPCPPCPAPEFLGGPSVFLFPPKPKDTLMISRTPEVTCVVVDVSQEDPEVQFNWYVDGVEVHNAKTKPREEQFNSTYRVVSVLTVLHQDWLNGKEYKCKVSNKGLPSSIEKTISKAKGQPREPQVYTLPPSQEEMTKNQVSLTCLVKGFYPSDIAVEWESNGQPENNYKTTPPVLDSDGSFFLYSRLTVDKSRWQEGNVFSCSVMHEALHNHYTQKSLSLSLGKEPKSSDKTHTSPPSPEVQLVESGGGLVQPGGSLRLSCAASGYIISSYCMGWFRQAPGKGLEGVAAIDSDGGTSYADSVKGRFTISKDNSKNTLYLQMNSLRAEDTAMYYCAADFCWVDEDRHLYEYNSWGQGTLVTVSS

SEQ ID NO: 386 - protein, 214 aa, Artificial Sequence; identical to SEQ ID NO: 374
  Synthetic Construct

SEQ ID NO: 387 - protein, 444 aa, Artificial Sequence; identical to SEQ ID NO: 373
  Synthetic Construct

SEQ ID NO: 388 - protein, 353 aa, Artificial Sequence
  Synthetic Construct
EVQLVESGGGLVQPGGSLRLSCAASGYIISSYCMGWFRQAPGKGLEGVAAIDSDGGTSYADSVKGRFTISKDNSKNTLYLQMNSLRAEDTAMYYCAADFCWVDEDRHLYEYNSWGQGTLVTVSSEPKSSDKTHTSPPSPDIQMTQSPSSVSASVGDRVTITCKASQDVDTAVAWYQQKPGKAPKLLIYWASTRHTGVPSRFSGSGSGTDFTLTISSLQPEDFATYYCQQYSTFPWTFGGGTKVEIKRTVAAPSVFIFPPSDEQLKSGTASVVCLLNNFYPREAKVQWKVDNALQSGNSQESVTEQDSKDSTYSLSSTLTLSKADYEKHKVYACEVTHQGLSSPVTKSFNRGEC

SEQ ID NO: 389 - protein, 444 aa, Artificial Sequence; identical to SEQ ID NO: 373
  Synthetic Construct

SEQ ID NO: 390 - protein, 353 aa, Artificial Sequence
  Synthetic Construct
DIQMTQSPSSVSASVGDRVTITCKASQDVDTAVAWYQQKPGKAPKLLIYWASTRHTGVPSRFSGSGSGTDFTLTISSLQPEDFATYYCQQYSTFPWTFGGGTKVEIKRTVAAPSVFIFPPSDEQLKSGTASVVCLLNNFYPREAKVQWKVDNALQSGNSQESVTEQDSKDSTYSLSSTLTLSKADYEKHKVYACEVTHQGLSSPVTKSFNRGECEPKSSDKTHTSPPSPEVQLVESGGGLVQPGGSLRLSCAASGYIISSYCMGWFRQAPGKGLEGVAAIDSDGGTSYADSVKGRFTISKDNSKNTLYLQMNSLRAEDTAMYYCAADFCWVDEDRHLYEYNSWGQGTLVTVSS

SEQ ID NO: 391 - protein, 580 aa, Artificial Sequence
  Synthetic Construct
EVQLVESGGGLVQPGGSLRLSCAASGYTISSYCMGWFRQAPGKGLEGVAAIDSDGSTSYADSVKGRFTISKDNSKNTLYLQMNSLRAEDTAVYYCAADFCWVDDFYEYNYWGQGTLVTVSSEPKSSDKTHTSPPSPEVQLVESGGGLVQPGGSLRLSCAASGFVFSRYDMAWVRQAPGKGLEWVSFISGGGSNTYYPDTVKGRFTISRDNSKNTLYLQMNSLRAEDTAVYYCISPYYYAMEYWGQGTTVTVSSASTKGPSVFPLAPCSRSTSESTAALGCLVKDYFPEPVTVSWNSGALTSGVHTFPAVLQSSGLYSLSSVVTVPSSSLGTKTYTCNVDHKPSNTKVDKRVESKYGPPCPPCPAPEFLGGPSVFLFPPKPKDTLMISRTPEVTCVVVDVSQEDPEVQFNWYVDGVEVHNAKTKPREEQFNSTYRVVSVLTVLHQDWLNGKEYKCKVSNKGLPSSIEKTISKAKGQPREPQVYTLPPSQEEMTKNQVSLTCLVKGFYPSDIAVEWESNGQPENNYKTTPPVLDSDGSFFLYSRLTVDKSRWQEGNVFSCSVMHEALHNHYTQKSLSLSLGK

SEQ ID NO: 392 - protein, 214 aa, Artificial Sequence; identical to SEQ ID NO: 374
  Synthetic Construct

SEQ ID NO: 393 - protein, 580 aa, Artificial Sequence
  Synthetic Construct
EVQLVESGGGLVQPGGSLRLSCAASGFVFSRYDMAWVRQAPGKGLEWVSFISGGGSNTYYPDTVKGRFTISRDNSKNTLYLQMNSLRAEDTAVYYCISPYYYAMEYWGQGTTVTVSSASTKGPSVFPLAPCSRSTSESTAALGCLVKDYFPEPVTVSWNSGALTSGVHTFPAVLQSSGLYSLSSVVTVPSSSLGTKTYTCNVDHKPSNTKVDKRVESKYGPPCPPCPAPEFLGGPSVFLFPPKPKDTLMISRTPEVTCVVVDVSQEDPEVQFNWYVDGVEVHNAKTKPREEQFNSTYRVVSVLTVLHQDWLNGKEYKCKVSNKGLPSSIEKTISKAKGQPREPQVYTLPPSQEEMTKNQVSLTCLVKGFYPSDIAVEWESNGQPENNYKTTPPVLDSDGSFFLYSRLTVDKSRWQEGNVFSCSVMHEALHNHYTQKSLSLSLGKEPKSSDKTHTSPPSPEVQLVESGGGLVQPGGSLRLSCAASGYTISSYCMGWFRQAPGKGLEGVAAIDSDGSTSYADSVKGRFTISKDNSKNTLYLQMNSLRAEDTAVYYCAADFCWVDDFYEYNYWGQGTLVTVSS

SEQ ID NO: 394 - protein, 214 aa, Artificial Sequence; identical to SEQ ID NO: 374
  Synthetic Construct

SEQ ID NO: 395 - protein, 444 aa, Artificial Sequence; identical to SEQ ID NO: 373
  Synthetic Construct

SEQ ID NO: 396 - protein, 350 aa, Artificial Sequence
  Synthetic Construct
EVQLVESGGGLVQPGGSLRLSCAASGYTISSYCMGWFRQAPGKGLEGVAAIDSDGSTSYADSVKGRFTISKDNSKNTLYLQMNSLRAEDTAVYYCAADFCWVDDFYEYNYWGQGTLVTVSSEPKSSDKTHTSPPSPDIQMTQSPSSVSASVGDRVTITCKASQDVDTAVAWYQQKPGKAPKLLIYWASTRHTGVPSRFSGSGSGTDFTLTISSLQPEDFATYYCQQYSTFPWTFGGGTKVEIKRTVAAPSVFIFPPSDEQLKSGTASVVCLLNNFYPREAKVQWKVDNALQSGNSQESVTEQDSKDSTYSLSSTLTLSKADYEKHKVYACEVTHQGLSSPVTKSFNRGEC

SEQ ID NO: 397 - protein, 444 aa, Artificial Sequence; identical to SEQ ID NO: 373
  Synthetic Construct

SEQ ID NO: 398 - protein, 350 aa, Artificial Sequence
  Synthetic Construct
DIQMTQSPSSVSASVGDRVTITCKASQDVDTAVAWYQQKPGKAPKLLIYWASTRHTGVPSRFSGSGSGTDFTLTISSLQPEDFATYYCQQYSTFPWTFGGGTKVEIKRTVAAPSVFIFPPSDEQLKSGTASVVCLLNNFYPREAKVQWKVDNALQSGNSQESVTEQDSKDSTYSLSSTLTLSKADYEKHKVYACEVTHQGLSSPVTKSFNRGECEPKSSDKTHTSPPSPEVQLVESGGGLVQPGGSLRLSCAASGYTISSYCMGWFRQAPGKGLEGVAAIDSDGSTSYADSVKGRFTISKDNSKNTLYLQMNSLRAEDTAVYYCAADFCWVDDFYEYNYWGQGTLVTVSS

SEQ ID NO: 399 - protein, 581 aa, Artificial Sequence
  Synthetic Construct
EVQLVESGGGLVQPGGSLRLSCAASGYTVSSYCMGWFRQAPGKGREGVSAIDSDGSVSYADSVKGRFTISKDNSKNTLYLQMNSLRAEDTAVYFCAADLCWVDQDQGEYNTWGQGTLVTVSSEPKSSDKTHTSPPSPEVQLVESGGGLVQPGGSLRLSCAASGFVFSRYDMAWVRQAPGKGLEWVSFISGGGSNTYYPDTVKGRFTISRDNSKNTLYLQMNSLRAEDTAVYYCISPYYYAMEYWGQGTTVTVSSASTKGPSVFPLAPCSRSTSESTAALGCLVKDYFPEPVTVSWNSGALTSGVHTFPAVLQSSGLYSLSSVVTVPSSSLGTKTYTCNVDHKPSNTKVDKRVESKYGPPCPPCPAPEFLGGPSVFLFPPKPKDTLMISRTPEVTCVVVDVSQEDPEVQFNWYVDGVEVHNAKTKPREEQFNSTYRVVSVLTVLHQDWLNGKEYKCKVSNKGLPSSIEKTISKAKGQPREPQVYTLPPSQEEMTKNQVSLTCLVKGFYPSDIAVEWESNGQPENNYKTTPPVLDSDGSFFLYSRLTVDKSRWQEGNVFSCSVMHEALHNHYTQKSLSLSLGK

SEQ ID NO: 400 - protein, 214 aa, Artificial Sequence; identical to SEQ ID NO: 374
  Synthetic Construct

SEQ ID NO: 401 - protein, 581 aa, Artificial Sequence
  Synthetic Construct
EVQLVESGGGLVQPGGSLRLSCAASGFVFSRYDMAWVRQAPGKGLEWVSFISGGGSNTYYPDTVKGRFTISRDNSKNTLYLQMNSLRAEDTAVYYCISPYYYAMEYWGQGTTVTVSSASTKGPSVFPLAPCSRSTSESTAALGCLVKDYFPEPVTVSWNSGALTSGVHTFPAVLQSSGLYSLSSVVTVPSSSLGTKTYTCNVDHKPSNTKVDKRVESKYGPPCPPCPAPEFLGGPSVFLFPPKPKDTLMISRTPEVTCVVVDVSQEDPEVQFNWYVDGVEVHNAKTKPREEQFNSTYRVVSVLTVLHQDWLNGKEYKCKVSNKGLPSSIEKTISKAKGQPREPQVYTLPPSQEEMTKNQVSLTCLVKGFYPSDIAVEWESNGQPENNYKTTPPVLDSDGSFFLYSRLTVDKSRWQEGNVFSCSVMHEALHNHYTQKSLSLSLGKEPKSSDKTHTSPPSPEVQLVESGGGLVQPGGSLRLSCAASGYTVSSYCMGWFRQAPGKGREGVSAIDSDGSVSYADSVKGRFTISKDNSKNTLYLQMNSLRAEDTAVYFCAADLCWVDQDQGEYNTWGQGTLVTVSS

SEQ ID NO: 402 - protein, 214 aa, Artificial Sequence; identical to SEQ ID NO: 374
  Synthetic Construct

SEQ ID NO: 403 - protein, 444 aa, Artificial Sequence; identical to SEQ ID NO: 373
  Synthetic Construct

SEQ ID NO: 404 - protein, 351 aa, Artificial Sequence
  Synthetic Construct
EVQLVESGGGLVQPGGSLRLSCAASGYTVSSYCMGWFRQAPGKGREGVSAIDSDGSVSYADSVKGRFTISKDNSKNTLYLQMNSLRAEDTAVYFCAADLCWVDQDQGEYNTWGQGTLVTVSSEPKSSDKTHTSPPSPDIQMTQSPSSVSASVGDRVTITCKASQDVDTAVAWYQQKPGKAPKLLIYWASTRHTGVPSRFSGSGSGTDFTLTISSLQPEDFATYYCQQYSTFPWTFGGGTKVEIKRTVAAPSVFIFPPSDEQLKSGTASVVCLLNNFYPREAKVQWKVDNALQSGNSQESVTEQDSKDSTYSLSSTLTLSKADYEKHKVYACEVTHQGLSSPVTKSFNRGEC

SEQ ID NO: 405 - protein, 444 aa, Artificial Sequence; identical to SEQ ID NO: 373
  Synthetic Construct

SEQ ID NO: 406 - protein, 351 aa, Artificial Sequence
  Synthetic Construct
DIQMTQSPSSVSASVGDRVTITCKASQDVDTAVAWYQQKPGKAPKLLIYWASTRHTGVPSRFSGSGSGTDFTLTISSLQPEDFATYYCQQYSTFPWTFGGGTKVEIKRTVAAPSVFIFPPSDEQLKSGTASVVCLLNNFYPREAKVQWKVDNALQSGNSQESVTEQDSKDSTYSLSSTLTLSKADYEKHKVYACEVTHQGLSSPVTKSFNRGECEPKSSDKTHTSPPSPEVQLVESGGGLVQPGGSLRLSCAASGYTVSSYCMGWFRQAPGKGREGVSAIDSDGSVSYADSVKGRFTISKDNSKNTLYLQMNSLRAEDTAVYFCAADLCWVDQDQGEYNTWGQGTLVTVSS

SEQ ID NO: 407 - protein, 585 aa, Artificial Sequence
  Synthetic Construct
EVQLVESGGGLVQPGGSLRLSCAASGYTYGGYCMGWFRQAPGKGLEGVSTINSDGSTNYADSVKGRFTISRDNSKNTLYLQMNSLRAEDTAVYYCAVDLAPCWVAGPIEAADFGYWGQGTLVTVSSEPKSSDKTHTSPPSPEVQLVESGGGLVQPGGSLRLSCAASGFVFSRYDMAWVRQAPGKGLEWVSFISGGGSNTYYPDTVKGRFTISRDNSKNTLYLQMNSLRAEDTAVYYCISPYYYAMEYWGQGTTVTVSSASTKGPSVFPLAPCSRSTSESTAALGCLVKDYFPEPVTVSWNSGALTSGVHTFPAVLQSSGLYSLSSVVTVPSSSLGTKTYTCNVDHKPSNTKVDKRVESKYGPPCPPCPAPEFLGGPSVFLFPPKPKDTLMISRTPEVTCVVVDVSQEDPEVQFNWYVDGVEVHNAKTKPREEQFNSTYRVVSVLTVLHQDWLNGKEYKCKVSNKGLPSSIEKTISKAKGQPREPQVYTLPPSQEEMTKNQVSLTCLVKGFYPSDIAVEWESNGQPENNYKTTPPVLDSDGSFFLYSRLTVDKSRWQEGNVFSCSVMHEALHNHYTQKSLSLSLGK

SEQ ID NO: 408 - protein, 214 aa, Artificial Sequence; identical to SEQ ID NO: 374
  Synthetic Construct

SEQ ID NO: 409 - protein, 585 aa, Artificial Sequence
  Synthetic Construct
EVQLVESGGGLVQPGGSLRLSCAASGFVFSRYDMAWVRQAPGKGLEWVSFISGGGSNTYYPDTVKGRFTISRDNSKNTLYLQMNSLRAEDTAVYYCISPYYYAMEYWGQGTTVTVSSASTKGPSVFPLAPCSRSTSESTAALGCLVKDYFPEPVTVSWNSGALTSGVHTFPAVLQSSGLYSLSSVVTVPSSSLGTKTYTCNVDHKPSNTKVDKRVESKYGPPCPPCPAPEFLGGPSVFLFPPKPKDTLMISRTPEVTCVVVDVSQEDPEVQFNWYVDGVEVHNAKTKPREEQFNSTYRVVSVLTVLHQDWLNGKEYKCKVSNKGLPSSIEKTISKAKGQPREPQVYTLPPSQEEMTKNQVSLTCLVKGFYPSDIAVEWESNGQPENNYKTTPPVLDSDGSFFLYSRLTVDKSRWQEGNVFSCSVMHEALHNHYTQKSLSLSLGKEPKSSDKTHTSPPSPEVQLVESGGGLVQPGGSLRLSCAASGYTYGGYCMGWFRQAPGKGLEGVSTINSDGSTNYADSVKGRFTISRDNSKNTLYLQMNSLRAEDTAVYYCAVDLAPCWVAGPIEAADFGYWGQGTLVTVSS

SEQ ID NO: 410 - protein, 214 aa, Artificial Sequence; identical to SEQ ID NO: 374
  Synthetic Construct

SEQ ID NO: 411 - protein, 444 aa, Artificial Sequence; identical to SEQ ID NO: 373
  Synthetic Construct

SEQ ID NO: 412 - protein, 355 aa, Artificial Sequence
  Synthetic Construct
EVQLVESGGGLVQPGGSLRLSCAASGYTYGGYCMGWFRQAPGKGLEGVSTINSDGSTNYADSVKGRFTISRDNSKNTLYLQMNSLRAEDTAVYYCAVDLAPCWVAGPIEAADFGYWGQGTLVTVSSEPKSSDKTHTSPPSPDIQMTQSPSSVSASVGDRVTITCKASQDVDTAVAWYQQKPGKAPKLLIYWASTRHTGVPSRFSGSGSGTDFTLTISSLQPEDFATYYCQQYSTFPWTFGGGTKVEIKRTVAAPSVFIFPPSDEQLKSGTASVVCLLNNFYPREAKVQWKVDNALQSGNSQESVTEQDSKDSTYSLSSTLTLSKADYEKHKVYACEVTHQGLSSPVTKSFNRGEC

SEQ ID NO: 413 - protein, 444 aa, Artificial Sequence; identical to SEQ ID NO: 373
  Synthetic Construct

SEQ ID NO: 414 - protein, 355 aa, Artificial Sequence
  Synthetic Construct
DIQMTQSPSSVSASVGDRVTITCKASQDVDTAVAWYQQKPGKAPKLLIYWASTRHTGVPSRFSGSGSGTDFTLTISSLQPEDFATYYCQQYSTFPWTFGGGTKVEIKRTVAAPSVFIFPPSDEQLKSGTASVVCLLNNFYPREAKVQWKVDNALQSGNSQESVTEQDSKDSTYSLSSTLTLSKADYEKHKVYACEVTHQGLSSPVTKSFNRGECEPKSSDKTHTSPPSPEVQLVESGGGLVQPGGSLRLSCAASGYTYGGYCMGWFRQAPGKGLEGVSTINSDGSTNYADSVKGRFTISRDNSKNTLYLQMNSLRAEDTAVYYCAVDLAPCWVAGPIEAADFGYWGQGTLVTVSS

SEQ ID NO: 415 - protein, 568 aa, Artificial Sequence
  Synthetic Construct
EVQLVESGGGLVQPGGSLRLSCAASGYIISSYCMGWFRQAPGKGLEGVAAIDSDGGTSYADSVKGRFTISKDNSKNTLYLQMNSLRAEDTAMYYCAADFCWVDEDRHLYEYNSWGQGTLVTVSSEVQLVESGGGLVQPGGSLRLSCAASGFVFSRYDMAWVRQAPGKGLEWVSFISGGGSNTYYPDTVKGRFTISRDNSKNTLYLQMNSLRAEDTAVYYCISPYYYAMEYWGQGTTVTVSSASTKGPSVFPLAPCSRSTSESTAALGCLVKDYFPEPVTVSWNSGALTSGVHTFPAVLQSSGLYSLSSVVTVPSSSLGTKTYTCNVDHKPSNTKVDKRVESKYGPPCPPCPAPEFLGGPSVFLFPPKPKDTLMISRTPEVTCVVVDVSQEDPEVQFNWYVDGVEVHNAKTKPREEQFNSTYRVVSVLTVLHQDWLNGKEYKCKVSNKGLPSSIEKTISKAKGQPREPQVYTLPPSQEEMTKNQVSLTCLVKGFYPSDIAVEWESNGQPENNYKTTPPVLDSDGSFFLYSRLTVDKSRWQEGNVFSCSVMHEALHNHYTQKSLSLSLGK

SEQ ID NO: 416 - protein, 214 aa, Artificial Sequence; identical to SEQ ID NO: 374
  Synthetic Construct

SEQ ID NO: 417 - protein, 444 aa, Artificial Sequence; identical to SEQ ID NO: 373
  Synthetic Construct

SEQ ID NO: 418 - protein, 338 aa, Artificial Sequence
  Synthetic Construct
EVQLVESGGGLVQPGGSLRLSCAASGYIISSYCMGWFRQAPGKGLEGVAAIDSDGGTSYADSVKGRFTISKDNSKNTLYLQMNSLRAEDTAMYYCAADFCWVDEDRHLYEYNSWGQGTLVTVSSDIQMTQSPSSVSASVGDRVTITCKASQDVDTAVAWYQQKPGKAPKLLIYWASTRHTGVPSRFSGSGSGTDFTLTISSLQPEDFATYYCQQYSTFPWTFGGGTKVEIKRTVAAPSVFIFPPSDEQLKSGTASVVCLLNNFYPREAKVQWKVDNALQSGNSQESVTEQDSKDSTYSLSSTLTLSKADYEKHKVYACEVTHQGLSSPVTKSFNRGEC

SEQ ID NO: 419 - protein, 565 aa, Artificial Sequence
  Synthetic Construct
EVQLVESGGGLVQPGGSLRLSCAASGYTISSYCMGWFRQAPGKGLEGVAAIDSDGSTSYADSVKGRFTISKDNSKNTLYLQMNSLRAEDTAVYYCAADFCWVDDFYEYNYWGQGTLVTVSSEVQLVESGGGLVQPGGSLRLSCAASGFVFSRYDMAWVRQAPGKGLEWVSFISGGGSNTYYPDTVKGRFTISRDNSKNTLYLQMNSLRAEDTAVYYCISPYYYAMEYWGQGTTVTVSSASTKGPSVFPLAPCSRSTSESTAALGCLVKDYFPEPVTVSWNSGALTSGVHTFPAVLQSSGLYSLSSVVTVPSSSLGTKTYTCNVDHKPSNTKVDKRVESKYGPPCPPCPAPEFLGGPSVFLFPPKPKDTLMISRTPEVTCVVVDVSQEDPEVQFNWYVDGVEVHNAKTKPREEQFNSTYRVVSVLTVLHQDWLNGKEYKCKVSNKGLPSSIEKTISKAKGQPREPQVYTLPPSQEEMTKNQVSLTCLVKGFYPSDIAVEWESNGQPENNYKTTPPVLDSDGSFFLYSRLTVDKSRWQEGNVFSCSVMHEALHNHYTQKSLSLSLGK

SEQ ID NO: 420 - protein, 214 aa, Artificial Sequence; identical to SEQ ID NO: 374
  Synthetic Construct

SEQ ID NO: 421 - protein, 444 aa, Artificial Sequence; identical to SEQ ID NO: 373
  Synthetic Construct

SEQ ID NO: 422 - protein, 335 aa, Artificial Sequence
  Synthetic Construct
EVQLVESGGGLVQPGGSLRLSCAASGYTISSYCMGWFRQAPGKGLEGVAAIDSDGSTSYADSVKGRFTISKDNSKNTLYLQMNSLRAEDTAVYYCAADFCWVDDFYEYNYWGQGTLVTVSSDIQMTQSPSSVSASVGDRVTITCKASQDVDTAVAWYQQKPGKAPKLLIYWASTRHTGVPSRFSGSGSGTDFTLTISSLQPEDFATYYCQQYSTFPWTFGGGTKVEIKRTVAAPSVFIFPPSDEQLKSGTASVVCLLNNFYPREAKVQWKVDNALQSGNSQESVTEQDSKDSTYSLSSTLTLSKADYEKHKVYACEVTHQGLSSPVTKSFNRGEC

SEQ ID NO: 423 - protein, 566 aa, Artificial Sequence
  Synthetic Construct
EVQLVESGGGLVQPGGSLRLSCAASGYTVSSYCMGWFRQAPGKGREGVSAIDSDGSVSYADSVKGRFTISKDNSKNTLYLQMNSLRAEDTAVYFCAADLCWVDQDQGEYNTWGQGTLVTVSSEVQLVESGGGLVQPGGSLRLSCAASGFVFSRYDMAWVRQAPGKGLEWVSFISGGGSNTYYPDTVKGRFTISRDNSKNTLYLQMNSLRAEDTAVYYCISPYYYAMEYWGQGTTVTVSSASTKGPSVFPLAPCSRSTSESTAALGCLVKDYFPEPVTVSWNSGALTSGVHTFPAVLQSSGLYSLSSVVTVPSSSLGTKTYTCNVDHKPSNTKVDKRVESKYGPPCPPCPAPEFLGGPSVFLFPPKPKDTLMISRTPEVTCVVVDVSQEDPEVQFNWYVDGVEVHNAKTKPREEQFNSTYRVVSVLTVLHQDWLNGKEYKCKVSNKGLPSSIEKTISKAKGQPREPQVYTLPPSQEEMTKNQVSLTCLVKGFYPSDIAVEWESNGQPENNYKTTPPVLDSDGSFFLYSRLTVDKSRWQEGNVFSCSVMHEALHNHYTQKSLSLSLGK

SEQ ID NO: 424 - protein, 214 aa, Artificial Sequence; identical to SEQ ID NO: 374
  Synthetic Construct

SEQ ID NO: 425 - protein, 444 aa, Artificial Sequence; identical to SEQ ID NO: 373
  Synthetic Construct

SEQ ID NO: 426 - protein, 336 aa, Artificial Sequence
  Synthetic Construct
EVQLVESGGGLVQPGGSLRLSCAASGYTVSSYCMGWFRQAPGKGREGVSAIDSDGSVSYADSVKGRFTISKDNSKNTLYLQMNSLRAEDTAVYFCAADLCWVDQDQGEYNTWGQGTLVTVSSDIQMTQSPSSVSASVGDRVTITCKASQDVDTAVAWYQQKPGKAPKLLIYWASTRHTGVPSRFSGSGSGTDFTLTISSLQPEDFATYYCQQYSTFPWTFGGGTKVEIKRTVAAPSVFIFPPSDEQLKSGTASVVCLLNNFYPREAKVQWKVDNALQSGNSQESVTEQDSKDSTYSLSSTLTLSKADYEKHKVYACEVTHQGLSSPVTKSFNRGEC

SEQ ID NO: 427 - protein, 570 aa, Artificial Sequence
  Synthetic Construct
EVQLVESGGGLVQPGGSLRLSCAASGYTYGGYCMGWFRQAPGKGLEGVSTINSDGSTNYADSVKGRFTISRDNSKNTLYLQMNSLRAEDTAVYYCAVDLAPCWVAGPIEAADFGYWGQGTLVTVSSEVQLVESGGGLVQPGGSLRLSCAASGFVFSRYDMAWVRQAPGKGLEWVSFISGGGSNTYYPDTVKGRFTISRDNSKNTLYLQMNSLRAEDTAVYYCISPYYYAMEYWGQGTTVTVSSASTKGPSVFPLAPCSRSTSESTAALGCLVKDYFPEPVTVSWNSGALTSGVHTFPAVLQSSGLYSLSSVVTVPSSSLGTKTYTCNVDHKPSNTKVDKRVESKYGPPCPPCPAPEFLGGPSVFLFPPKPKDTLMISRTPEVTCVVVDVSQEDPEVQFNWYVDGVEVHNAKTKPREEQFNSTYRVVSVLTVLHQDWLNGKEYKCKVSNKGLPSSIEKTISKAKGQPREPQVYTLPPSQEEMTKNQVSLTCLVKGFYPSDIAVEWESNGQPENNYKTTPPVLDSDGSFFLYSRLTVDKSRWQEGNVFSCSVMHEALHNHYTQKSLSLSLGK

SEQ ID NO: 428 - protein, 214 aa, Artificial Sequence; identical to SEQ ID NO: 374
  Synthetic Construct

SEQ ID NO: 429 - protein, 444 aa, Artificial Sequence; identical to SEQ ID NO: 373
  Synthetic Construct

SEQ ID NO: 430 - protein, 340 aa, Artificial Sequence
  Synthetic Construct
EVQLVESGGGLVQPGGSLRLSCAASGYTYGGYCMGWFRQAPGKGLEGVSTINSDGSTNYADSVKGRFTISRDNSKNTLYLQMNSLRAEDTAVYYCAVDLAPCWVAGPIEAADFGYWGQGTLVTVSSDIQMTQSPSSVSASVGDRVTITCKASQDVDTAVAWYQQKPGKAPKLLIYWASTRHTGVPSRFSGSGSGTDFTLTISSLQPEDFATYYCQQYSTFPWTFGGGTKVEIKRTVAAPSVFIFPPSDEQLKSGTASVVCLLNNFYPREAKVQWKVDNALQSGNSQESVTEQDSKDSTYSLSSTLTLSKADYEKHKVYACEVTHQGLSSPVTKSFNRGEC

SEQ ID NO: 431 - protein, 583 aa, Artificial Sequence
  Synthetic Construct
EPKSSDKTHTSPPSPEVQLVESGGGLVQPGGSLRLSCAASGYIISSYCMGWFRQAPGKGLEGVAAIDSDGGTSYADSVKGRFTISKDNSKNTLYLQMNSLRAEDTAMYYCAADFCWVDEDRHLYEYNSWGQGTLVTVSSEVQLVESGGGLVQPGGSLRLSCAASGFVFSRYDMAWVRQAPGKGLEWVSFISGGGSNTYYPDTVKGRFTISRDNSKNTLYLQMNSLRAEDTAVYYCISPYYYAMEYWGQGTTVTVSSASTKGPSVFPLAPCSRSTSESTAALGCLVKDYFPEPVTVSWNSGALTSGVHTFPAVLQSSGLYSLSSVVTVPSSSLGTKTYTCNVDHKPSNTKVDKRVESKYGPPCPPCPAPEFLGGPSVFLFPPKPKDTLMISRTPEVTCVVVDVSQEDPEVQFNWYVDGVEVHNAKTKPREEQFNSTYRVVSVLTVLHQDWLNGKEYKCKVSNKGLPSSIEKTISKAKGQPREPQVYTLPPSQEEMTKNQVSLTCLVKGFYPSDIAVEWESNGQPENNYKTTPPVLDSDGSFFLYSRLTVDKSRWQEGNVFSCSVMHEALHNHYTQKSLSLSLGK

SEQ ID NO: 432 - protein, 214 aa, Artificial Sequence; identical to SEQ ID NO: 374
  Synthetic Construct

SEQ ID NO: 433 - protein, 444 aa, Artificial Sequence; identical to SEQ ID NO: 373
  Synthetic Construct

SEQ ID NO: 434 - protein, 353 aa, Artificial Sequence
  Synthetic Construct
EPKSSDKTHTSPPSPEVQLVESGGGLVQPGGSLRLSCAASGYIISSYCMGWFRQAPGKGLEGVAAIDSDGGTSYADSVKGRFTISKDNSKNTLYLQMNSLRAEDTAMYYCAADFCWVDEDRHLYEYNSWGQGTLVTVSSDIQMTQSPSSVSASVGDRVTITCKASQDVDTAVAWYQQKPGKAPKLLIYWASTRHTGVPSRFSGSGSGTDFTLTISSLQPEDFATYYCQQYSTFPWTFGGGTKVEIKRTVAAPSVFIFPPSDEQLKSGTASVVCLLNNFYPREAKVQWKVDNALQSGNSQESVTEQDSKDSTYSLSSTLTLSKADYEKHKVYACEVTHQGLSSPVTKSFNRGEC

SEQ ID NO: 435 - protein, 580 aa, Artificial Sequence
  Synthetic Construct
EPKSSDKTHTSPPSPEVQLVESGGGLVQPGGSLRLSCAASGYTISSYCMGWFRQAPGKGLEGVAAIDSDGSTSYADSVKGRFTISKDNSKNTLYLQMNSLRAEDTAVYYCAADFCWVDDFYEYNYWGQGTLVTVSSEVQLVESGGGLVQPGGSLRLSCAASGFVFSRYDMAWVRQAPGKGLEWVSFISGGGSNTYYPDTVKGRFTISRDNSKNTLYLQMNSLRAEDTAVYYCISPYYYAMEYWGQGTTVTVSSASTKGPSVFPLAPCSRSTSESTAALGCLVKDYFPEPVTVSWNSGALTSGVHTFPAVLQSSGLYSLSSVVTVPSSSLGTKTYTCNVDHKPSNTKVDKRVESKYGPPCPPCPAPEFLGGPSVFLFPPKPKDTLMISRTPEVTCVVVDVSQEDPEVQFNWYVDGVEVHNAKTKPREEQFNSTYRVVSVLTVLHQDWLNGKEYKCKVSNKGLPSSIEKTISKAKGQPREPQVYTLPPSQEEMTKNQVSLTCLVKGFYPSDIAVEWESNGQPENNYKTTPPVLDSDGSFFLYSRLTVDKSRWQEGNVFSCSVMHEALHNHYTQKSLSLSLGK

SEQ ID NO: 436 - protein, 214 aa, Artificial Sequence; identical to SEQ ID NO: 374
  Synthetic Construct

SEQ ID NO: 437 - protein, 444 aa, Artificial Sequence; identical to SEQ ID NO: 373
  Synthetic Construct

SEQ ID NO: 438 - protein, 350 aa, Artificial Sequence
  Synthetic Construct
EPKSSDKTHTSPPSPEVQLVESGGGLVQPGGSLRLSCAASGYTISSYCMGWFRQAPGKGLEGVAAIDSDGSTSYADSVKGRFTISKDNSKNTLYLQMNSLRAEDTAVYYCAADFCWVDDFYEYNYWGQGTLVTVSSDIQMTQSPSSVSASVGDRVTITCKASQDVDTAVAWYQQKPGKAPKLLIYWASTRHTGVPSRFSGSGSGTDFTLTISSLQPEDFATYYCQQYSTFPWTFGGGTKVEIKRTVAAPSVFIFPPSDEQLKSGTASVVCLLNNFYPREAKVQWKVDNALQSGNSQESVTEQDSKDSTYSLSSTLTLSKADYEKHKVYACEVTHQGLSSPVTKSFNRGEC

SEQ ID NO: 439 - protein, 581 aa, Artificial Sequence
  Synthetic Construct
EPKSSDKTHTSPPSPEVQLVESGGGLVQPGGSLRLSCAASGYTVSSYCMGWFRQAPGKGREGVSAIDSDGSVSYADSVKGRFTISKDNSKNTLYLQMNSLRAEDTAVYFCAADLCWVDQDQGEYNTWGQGTLVTVSSEVQLVESGGGLVQPGGSLRLSCAASGFVFSRYDMAWVRQAPGKGLEWVSFISGGGSNTYYPDTVKGRFTISRDNSKNTLYLQMNSLRAEDTAVYYCISPYYYAMEYWGQGTTVTVSSASTKGPSVFPLAPCSRSTSESTAALGCLVKDYFPEPVTVSWNSGALTSGVHTFPAVLQSSGLYSLSSVVTVPSSSLGTKTYTCNVDHKPSNTKVDKRVESKYGPPCPPCPAPEFLGGPSVFLFPPKPKDTLMISRTPEVTCVVVDVSQEDPEVQFNWYVDGVEVHNAKTKPREEQFNSTYRVVSVLTVLHQDWLNGKEYKCKVSNKGLPSSIEKTISKAKGQPREPQVYTLPPSQEEMTKNQVSLTCLVKGFYPSDIAVEWESNGQPENNYKTTPPVLDSDGSFFLYSRLTVDKSRWQEGNVFSCSVMHEALHNHYTQKSLSLSLGK

SEQ ID NO: 440 - protein, 214 aa, Artificial Sequence; identical to SEQ ID NO: 374
  Synthetic Construct

SEQ ID NO: 441 - protein, 444 aa, Artificial Sequence; identical to SEQ ID NO: 373
  Synthetic Construct

SEQ ID NO: 442 - protein, 351 aa, Artificial Sequence
  Synthetic Construct
EPKSSDKTHTSPPSPEVQLVESGGGLVQPGGSLRLSCAASGYTVSSYCMGWFRQAPGKGREGVSAIDSDGSVSYADSVKGRFTISKDNSKNTLYLQMNSLRAEDTAVYFCAADLCWVDQDQGEYNTWGQGTLVTVSSDIQMTQSPSSVSASVGDRVTITCKASQDVDTAVAWYQQKPGKAPKLLIYWASTRHTGVPSRFSGSGSGTDFTLTISSLQPEDFATYYCQQYSTFPWTFGGGTKVEIKRTVAAPSVFIFPPSDEQLKSGTASVVCLLNNFYPREAKVQWKVDNALQSGNSQESVTEQDSKDSTYSLSSTLTLSKADYEKHKVYACEVTHQGLSSPVTKSFNRGEC

SEQ ID NO: 443 - protein, 585 aa, Artificial Sequence
  Synthetic Construct
EPKSSDKTHTSPPSPEVQLVESGGGLVQPGGSLRLSCAASGYTYGGYCMGWFRQAPGKGLEGVSTINSDGSTNYADSVKGRFTISRDNSKNTLYLQMNSLRAEDTAVYYCAVDLAPCWVAGPIEAADFGYWGQGTLVTVSSEVQLVESGGGLVQPGGSLRLSCAASGFVFSRYDMAWVRQAPGKGLEWVSFISGGGSNTYYPDTVKGRFTISRDNSKNTLYLQMNSLRAEDTAVYYCISPYYYAMEYWGQGTTVTVSSASTKGPSVFPLAPCSRSTSESTAALGCLVKDYFPEPVTVSWNSGALTSGVHTFPAVLQSSGLYSLSSVVTVPSSSLGTKTYTCNVDHKPSNTKVDKRVESKYGPPCPPCPAPEFLGGPSVFLFPPKPKDTLMISRTPEVTCVVVDVSQEDPEVQFNWYVDGVEVHNAKTKPREEQFNSTYRVVSVLTVLHQDWLNGKEYKCKVSNKGLPSSIEKTISKAKGQPREPQVYTLPPSQEEMTKNQVSLTCLVKGFYPSDIAVEWESNGQPENNYKTTPPVLDSDGSFFLYSRLTVDKSRWQEGNVFSCSVMHEALHNHYTQKSLSLSLGK

SEQ ID NO: 444 - protein, 214 aa, Artificial Sequence; identical to SEQ ID NO: 374
  Synthetic Construct

SEQ ID NO: 445 - protein, 444 aa, Artificial Sequence; identical to SEQ ID NO: 373
  Synthetic Construct

SEQ ID NO: 446 - protein, 355 aa, Artificial Sequence
  Synthetic Construct
EPKSSDKTHTSPPSPEVQLVESGGGLVQPGGSLRLSCAASGYTYGGYCMGWFRQAPGKGLEGVSTINSDGSTNYADSVKGRFTISRDNSKNTLYLQMNSLRAEDTAVYYCAVDLAPCWVAGPIEAADFGYWGQGTLVTVSSDIQMTQSPSSVSASVGDRVTITCKASQDVDTAVAWYQQKPGKAPKLLIYWASTRHTGVPSRFSGSGSGTDFTLTISSLQPEDFATYYCQQYSTFPWTFGGGTKVEIKRTVAAPSVFIFPPSDEQLKSGTASVVCLLNNFYPREAKVQWKVDNALQSGNSQESVTEQDSKDSTYSLSSTLTLSKADYEKHKVYACEVTHQGLSSPVTKSFNRGEC